European Patent Specification EP 3 585 910 B1, published March 20, 2024. Title: COMPOSITIONS AND METHODS FOR INCREASED PROTEIN PRODUCTION IN BACILLUS LICHENIFORMIS. Applicant: Danisco. The sequence listing filed with the application follows.

SEQUENCE LISTING (144 sequences)

SEQ ID NO: 1 - DNA, 405 bp, Bacillus licheniformis
atggcgatgacaaggttcggcgagcggctcaaagagctgagggaacaaagaagcctgtcggttaatcagcttgccatgtatgccggtgtgagcgccgcagccatttccagaatcgaaaacggccaccgcggcgttcccaagcccgcgacgatcagaaaattggccgaggctctgaaaatgccgtacgagcagctcatggatattgccggttatatgagagctgacgagattcgcgaacagccgcgcggctatgtcacgatgcaggagatcgcggccaagcacggcgtcgaagacctgtggctgtttaaacccgagaaatgggactgtttgtcccgcgaagacctgctcaacctcgaacagtattttcattttttggttaatgaagcgaagaagcgccaatcataa

SEQ ID NO: 2 - protein, 134 aa, Bacillus licheniformis
MAMTRFGERLKELREQRSLSVNQLAMYAGVSAAAISRIENGHRGVPKPATIRKLAEALKMPYEQLMDIAGYMRADEIREQPRGYVTMQEIAAKHGVEDLWLFKPEKWDCLSREDLLNLEQYFHFLVNEAKKRQS

SEQ ID NO: 3 - DNA, 423 bp, Bacillus licheniformis
atggcgatgacaaggttcggcgagcggctcaaagagctgagggaacaaagaagcctgtcggttaatcagcttgccatgtatgccggtgtgagcgccgcagccatttccagagccgcagccatttccagaatcgaaaacggccaccgcggcgttcccaagcccgcgacgatcagaaaattggccgaggctctgaaaatgccgtacgagcagctcatggatattgccggttatatgagagctgacgagattcgcgaacagccgcgcggctatgtcacgatgcaggagatcgcggccaagcacggcgtcgaagacctgtggctgtttaaacccgagaaatgggactgtttgtcccgcgaagacctgctcaacctcgaacagtattttcattttttggttaatgaagcgaagaagcgccaatcataa

SEQ ID NO: 4 - protein, 140 aa, Bacillus licheniformis
MAMTRFGERLKELREQRSLSVNQLAMYAGVSAAAISRAAAISRIENGHRGVPKPATIRKLAEALKMPYEQLMDIAGYMRADEIREQPRGYVTMQEIAAKHGVEDLWLFKPEKWDCLSREDLLNLEQYFHFLVNEAKKRQS

SEQ ID NO: 5 - protein, 6 aa, Bacillus licheniformis
AAAISR

SEQ ID NO: 6 - protein, 12 aa, Bacillus licheniformis
AAAISRAAAISR

SEQ ID NO: 7 - DNA, 26 bp, Artificial Sequence
  primer
gagactagtgagctcgcatcacacgc

SEQ ID NO: 8 - DNA, 38 bp, Artificial Sequence
  primer
gactgcggccgcaccatgattactcccctttctaatct

SEQ ID NO: 9 - DNA, 38 bp, Artificial Sequence
  primer
tctggaaatggctgcggcgctcacaccggcatacatgg

SEQ ID NO: 10 - DNA, 38 bp, Artificial Sequence
  primer
gccgcagccatttccagaatcgaaaacggccaccgcgg

SEQ ID NO: 11 - DNA, 28 bp, Artificial Sequence
  primer
gactaagcttcgccgtcttgatgcttgt

SEQ ID NO: 12 - DNA, 21 bp, Artificial Sequence
  primer
gtacggcattttcagagcctc

SEQ ID NO: 13 - DNA, 26 bp, Artificial Sequence
  primer
tgaatcatctttccgatcacaagttg

SEQ ID NO: 14 - DNA, 23 bp, Artificial Sequence
  primer
aaggaggggatgacaaatggaag

SEQ ID NO: 15 - DNA, 402 bp, Bacillus licheniformis
atgacgaactttggacaccatttacgacaattaagggaacggaaaaaactgaccgtcaatcaactggcgatgtattccggcgtcagttcggcaggcatttcgcgaatcgaaaacggaaagcgcggcgtgccgaagccggcgacgatcagaaaactggcggacgctttgaaagtcccgtatgaggaactgatggcatctgcaggctatatcagcgcgtctacagtccaggaagcaagaagcagctatgattccatttacgacatcgtgtcacagtacgatttagaggacctttctctgtttgacagcgaaaagtggaaggtgctttcaaaaaaagacatcgaaaacctggacaaatatttcgactttctcgtgcaggaagcaagcagccgaaacaaaaactga

SEQ ID NO: 16 - protein, 60 aa, Bacillus licheniformis
MTNFGHHLRQLRERKKLTVNQLAMYSGVSSAGISRIENGKRGVPKPATIRKLADALKVPY

SEQ ID NO: 17 - DNA, 231 bp, Bacillus licheniformis
atggtaaaaaagattcatatcaaaagagattttgttctccagtacatgattgaacacaatctctccttaaatcagcttgccattgaaatcggcgtatccccggcgacactcagcagagttttaaatggcgaaaggaggcccggacaacttgtgatcggaaagatgattcagtatttcaacaaaaaatttgaagatctcttttattataaagatgttgacaaaagtcaataa

SEQ ID NO: 18 - protein, 75 aa, Bacillus licheniformis
MVKKIHIKRDFVLQYMIEHNLSLNQLAIEIGVSPATLSRVLNGERRPGQLVIGKMIQYFNKKFEDLFYYKDVDKS

SEQ ID NO: 19 - DNA, 285 bp, Bacillus licheniformis
gtgaaaaataccgggattgtccggagaatcgatgagctcggcagagtcgttctcccggtcgaaatgcgcagggtgctgaatatcaatgaaaaggacccgctcgaaatatataccgacggcgaaaacatcattttgacaaaatacgccgcaaacatggcatgtttgatgaccggcgacatcaccacgaaaaataaaacgtatgcgggcggcaaaatcgtactcagcccgcgcggagcggaaatgctcctggaagatatgatggcggcactgtcagaaaagaaataa

SEQ ID NO: 20 - protein, 93 aa, Bacillus licheniformis
MKNTGIVRRIDELGRVVLPVEMRRVLNINEKDPLEIYTDGENIILTKYAANMACLMTGDITTKNKTYAGGKIVLSPRGAEMLLEDMMAALSEK

SEQ ID NO: 21 - DNA, 285 bp, Bacillus licheniformis
atgaaatctacaggtattgtacgtaaagttgatgaactaggacgcgtggtgattccaatcgaacttcgccgtacgcttggaatcgcagaaaaagacgctcttgaaatctatgtagatgacgaaaaaatcatcttgaaaaaatataaaccaaacatgacttgccaagttacaggtgaggtttctgatgacaaccttaaacttgcaggcggtaaattggttcttagccctgaaggcgctgagcaaatcattaacgaaattcaagcacaacttcaatctcaaaaataa

SEQ ID NO: 22 - protein, 94 aa, Bacillus licheniformis
MKSTGIVRKVDELGRVVIPIELRRTLGIAEKDALEIYVDDEKIILKKYKPNMTCQVTGEVSDDNLKLAGGKLVLSPEGAEQIINEIQAQLQSQK

SEQ ID NO: 23 - DNA, 288 bp, Bacillus licheniformis
ttgaaagcaataggagttgtgagaaaagtagacgaactcggcaggatcgtgatgccgattgaattgagaagagctttggatatctcgatcaaggacagcatcgaattctttgtcgaccaagataaaatcgtcctgaaaaaatataaaccgcacggtgtgtgtctgatgaccggtgaaatcacttctgaaaaccgcgagtatggaaacgggaaaattacgctcagtcctgaaggggccgaattgcttttggaagaaatcaaagctgccttaaacggagtgaaagcataa

SEQ ID NO: 24 - protein, 95 aa, Bacillus licheniformis
MKAIGVVRKVDELGRIVMPIELRRALDISIKDSIEFFVDQDKIVLKKYKPHGVCLMTGEITSENREYGNGKITLSPEGAELLLEEIKAALNGVKA

SEQ ID NO: 25 - DNA, 114 bp, Bacillus licheniformis
atgaaagtgagaccatcagttaaaccgatctgtgaaaaatgcaaggtcattcgcagaaaaggaaaagtaatggtgatctgtgaaaatccaaagcataaacaaaaacaaggataa

SEQ ID NO: 26 - protein, 37 aa, Bacillus licheniformis
MKVRPSVKPICEKCKVIRRKGKVMVICENPKHKQKQG

SEQ ID NO: 27 - DNA, 431 bp, Bacillus licheniformis
atgcgtacaacacctatggctaacgcaagtaatattgaacgcaagtggttagttgttgatgctgctggcaagacgctaggacgtctttctactgaagttgcatctatccttcgcggaaaacataaaccaacttacacaccacacgttgacactggagatcatgtgatcatcatcaacgctgaaaaaatcgagttaactggtaaaaagttaacggacaaaatctactaccgtcacactcaacatccaggcggtttaaaatcaagaactgctcttgaaatgcgtacaaactaccctgagaaaatgcttgaacttgcgatcaaaggcatgcttccaaaaggttctctaggtcgtcaaatgttcaaaaaattgaatgtataccgtggttctgagcatccacaccaagcacaaaaacctgaagtttacgaacttcg

SEQ ID NO: 28 - protein, 143 aa, Bacillus licheniformis
MRTTPMANASNIERKWLVVDAAGKTLGRLSTEVASILRGKHKPTYTPHVDTGDHVIIINAEKIELTGKKLTDKIYYRHTQHPGGLKSRTALEMRTNYPEKMLELAIKGMLPKGSLGRQMFKKLNVYRGSEHPHQAQKPEVYEL

SEQ ID NO: 29 - DNA, 915 bp, Bacillus licheniformis
atgggtacaatagggataaactttaaaaacattcaacatcaatatcgtaccaaggatgtgctaaggggggtgagtttccatgccgatccctcctccatcacgttcttggcaggcgagaatggagccggaaagacaactttgataaaggttgctctcggcttaatcagtccgaaggcaggaaatgcgctgttcgacgggcaaagcgtcggggaaatccgggagaagatcagctgcgtgtttgatgagcctcctgtttatcctaatgaaagtggtcttgacaatctaaagtttttatcaggtatacacagccttgatcgaaagtggagtcaggaggtttgtgccatgctcaaattggatgagggacttttaaaacaaaaagcaaaagcgctatcactgggtcaaagacaccgtttagctgtagcggccgcgttattgcgcaaacctaaatatttgtttcttgatgagccgtcaatcggcctcgacccaccgtcatggcagctggtccaaatcgctttaaaacagatgactgccaggggatgtgcaattttgattacggggcaaaattatgacgcgattgaaaatctcgctgacaatatagcgattttgcaaagtggaaaaattatcttctccggtcctattgtaaaacttgttcaagcatttcccgtatatgttcgaattgtaactgatgaccatcgggaaatagctgtgcagtttccagaagctgaacctgattcttccggaatataccgcatcgtttgcgaatcaggtgaacaggcccgcgccgtgattgatcaggtgaggagaagcaccctgaattttcaagagctatcgactgaaaaagcgtcaatggggaaaatggtgacagatatttacaaggatggatttcagtcggaaaagagagggttaacgtatgaa

SEQ ID NO: 30 - protein, 304 aa, Bacillus licheniformis
MGTIGINFKNIQHQYRTKDVLRGVSFHADPSSITFLAGENGAGKTTLIKVALGLISPKAGNALFDGQSVGEIREKISCVFDEPPVYPNESGLDNLKFLSGIHSLDRKWSQEVCAMLKLDEGLLKQKAKALSLGQRHRLAVAAALLRKPKYLFLDEPSIGLDPPSWQLVQIALKQMTARGCAILITGQNYDAIENLADNIAILQSGKIIFSGPIVKLVQAFPVYVRIVTDDHREIAVQFPEAEPDSSGIYRIVCESGEQARAVIDQVRRSTLNFQELSTEKASMGKMVTDIYKDGFQSEKRGLTY

SEQ ID NO: 31 - DNA, 1096 bp, Bacillus licheniformis
atgagcaaggtcgcttcagaggtggttgcgggggtgttgaacgaattccatttggccattaaaaagcacgatactgagcaggcaaagcatctttttgatgaggcgaagtcgatgttttccgagatggaagaggatcagaatgtgctggcttatttttcgcttcttgaggagcggtaccggatgatgctttatgatgcgaggggagagcggctgccgcgggagtcttattttaatgattcgcagatcgagtgcatcgagcagacggatcatatgattgattactatttctacttttttgaggcgatgcatgaagcgtacaacaagaatgttgagcgggcgatcagtctgtacaaggttgccgagaaaaaactggcgaaggtgcccgatcagattgaagcggccgagttttattttaaagtgtcctggctgtatatgtctcttcggcaaaatgcggtttctctcaattatgcgagagacgcgatgaatatttacaaaatgcatgacgggtacgaaaaaaagctggcgatttcccaagttgtgatggggacaaattacatgcagatgcagcgctttaaagatgcggagaagtactttgaagaatcgattgaaatttccaaaaagattgacgattcatttttagaagcgatgcttcatcacaatatcagcattctgtattccaattccggccggtctcaggaatgcattctcgccgtccagcatgctttgagcaacgccgaatggtgcaagtcaagctactatatcaactcgctttacatgctgaccagagagtttttcaaaatcggcgaaacagaagcggccctgttctatcataaaaaaggacaggaggaattaaagaaaaacgggaataagcattatgaaaagaaaataaatattatttatgagctgtattgccatgaaaacgtaaaaagcatcaaagacgacatccattccttggacgagatgaatgatttagacggtgtctgcgatctttctttgctcatctcaagctattttgagaaaaaaggagatgacaagaaagcgctggaatttgttaaaatattcatgaaagccgaaaacaaaatgagatcattaggga

SEQ ID NO: 32 - protein, 364 aa, Bacillus licheniformis
MSKVASEVVAGVLNEFHLAIKKHDTEQAKHLFDEAKSMFSEMEEDQNVLAYFSLLEERYRMMLYDARGERLPRESYFNDSQIECIEQTDHMIDYYFYFFEAMHEAYNKNVERAISLYKVAEKKLAKVPDQIEAAEFYFKVSWLYMSLRQNAVSLNYARDAMNIYKMHDGYEKKLAISQVVMGTNYMQMQRFKDAEKYFEESIEISKKIDDSFLEAMLHHNISILYSNSGRSQECILAVQHALSNAEWCKSSYYINSLYMLTREFFKIGETEAALFYHKKGQEELKKNGNKHYEKKINIIYELYCHENVKSIKDDIHSLDEMNDLDGVCDLSLLISSYFEKKGDDKKALEFVKIFMKAENKMRSL

SEQ ID NO: 33 - DNA, 121 bp, Bacillus licheniformis
atgaaaaaattaattctttgcttgtcgttaactgctatggtcttaggcggagctgctttatcccaaagccacaatcaggcgtcaggcggcgttcaaacagcggagctgccggttgggggtt

SEQ ID NO: 34 - protein, 40 aa, Bacillus licheniformis
MKKLILCLSLTAMVLGGAALSQSHNQASGGVQTAELPVGG

SEQ ID NO: 35 - DNA, 747 bp, Bacillus licheniformis
atgaatgacaaaacatttttatcatttttaaaacacgcagataagcctttcagcggctgggatttttctttcattgaagacacaggacgaatgaaaagcgacctgctttcatggtcatacggaagcatggctctgtctcttatccaggattccgaatcaatgttggatatggggacaggcggcggcgagtttttatccaaattggggccgtttccttcgtcagcatacgctactgaatgttatttgcctaatgtgccagtcgccaaggaacgattgacgcctttaggggttcaggtcgttcaaattgatgatgatgaagatcttccatttgaatccggccaattcgacctgatcatcaataaacacgaatcatattcagtacaagaggtgaggagaatcctttcaaaaggaggacggtttctcactcagcaagtcggcgggcttgattgcgaagaaataaatgaaaaacttggcgtgccgctaaatgaagaatttaaggattgggacttggaaacagcgttaaaagagatggaaaagcatgattttaagattttaaaaagcagagaagagtgtccgactcaaaggttttatgatattggggctctggtctattatttgaaagccattccctggcaggcgctcggttttgaagtgaatcaatataaggatgaattgtacgagattcataaaatgatcgaagaaaagggctattttgacgtcacacagtaccggtttatgattttagcg

SEQ ID NO: 36 - protein, 248 aa, Bacillus licheniformis
MNDKTFLSFLKHADKPFSGWDFSFIEDTGRMKSDLLSWSYGSMALSLIQDSESMLDMGTGGGEFLSKLGPFPSSAYATECYLPNVPVAKERLTPLGVQVVQIDDDEDLPFESGQFDLIINKHESYSVQEVRRILSKGGRFLTQQVGGLDCEEINEKLGVPLNEEFKDWDLETALKEMEKHDFKILKSREECPTQRFYDIGALVYYLKAIPWQALGFEVNQYKDELYEIHKMIEEKGYFDVTQYRFMIL

SEQ ID NO: 37 - DNA, 183 bp, Bacillus licheniformis
atgggtaacgcagtacatgacaaagaacagcaagtcaattatttgaaaaacagattggatatgtttatgtcagtcatcgattctttagacccggaatcgaccgaccttgaagatattgacagactgatcagcatgctcgacgatttggaagccaaatacgagcgctttaaaaaagactggaaa

SEQ ID NO: 38 - protein, 61 aa, Bacillus licheniformis
MGNAVHDKEQQVNYLKNRLDMFMSVIDSLDPESTDLEDIDRLISMLDDLEAKYERFKKDWK

SEQ ID NO: 39 - DNA, 1086 bp, Bacillus licheniformis
atgtcaaaatcagtaaaatcagtcacatcacctaaaaaatttattacaggaaaacgactgctggagaacttgaacgactacattgaagattttggcgacaacgcatatatcatttgcgatgaattcattttggaacgcgctcaaaaagaagcggggaattcgattcagaaagccggcaatcaagccgtttttgaaaaattcaattacgaatgcacacaggaagaaatcgatcgcaaccgggagcttgcacgcaatgcaggcgctaatatcatcgttgggatcggaggcggtaaaacgcttgataccgcaaaagccaccgcttattacgagaagctgccggttgtgattttcccgacaattgcttctacggatgctccatgtacggcccttgccgtcatttataaacacgacggatcgtttgaccgctatctgtttttgccgacgaacccagatgtcgttcttgcggactctgagattttggcatccgcgccgccgcgctttttcgcagccggtatcggtgacgccttggcgacgtattttgaagcgcgtgcctgctttaaagcaaacggcgataacctcgtgctgatgaagccttcaacaactggattgggacttgcccgtctttgctatgatacgctgttggaaaacggtgtgaaagcgatgcaggcggttaagcacggcgtttccacacgagcggtcgaagatacaatcgaggcgaccatctatttaagcggcgtcggtgccgaatcaggcggtcttgccgccgcacacgcgatccacaacggaatgacagccgttccttctctgcacagggctcagcacggcgaaaaagtcacgttcggccttttggcgcagcttgttcttgaaaacgcgccggccgaagaattggagaccgttattgactttatcaaaggcgtcggtcttccgttgacattaaaagacctcggagtcgacgaatttgtcgaagaagaatggcgccaagtcgctcaaagcgcttgcgcggaaggcgacacaatgggcaacatgccgttcccagtcacccctgacgacgtctacaatgcgatcgtcgccgccaacgcgattgca

SEQ ID NO: 40 - protein, 361 aa, Bacillus licheniformis
MSKSVKSVTSPKKFITGKRLLENLNDYIEDFGDNAYIICDEFILERAQKEAGNSIQKAGNQAVFEKFNYECTQEEIDRNRELARNAGANIIVGIGGGKTLDTAKATAYYEKLPVVIFPTIASTDAPCTALAVIYKHDGSFDRYLFLPTNPDVVLADSEILASAPPRFFAAGIGDALATYFEARACFKANGDNLVLMKPSTTGLGLARLCYDTLLENGVKAMQAVKHGVSTRAVEDTIEATIYLSGVGAESGGLAAAHAIHNGMTAVPSLHRAQHGEKVTFGLLAQLVLENAPAEELETVIDFIKGVGLPLTLKDLGVDEFVEEEWRQVAQSACAEGDTMGNMPFPVTPDDVYNAIVAANAI

SEQ ID NO: 41 - DNA, 110 bp, Bacillus licheniformis
atgatgggtaaagggagaattaaagtggaagaacggattaagatcgaaaccgatgctgaaatgtttaaagcgactctccttgatcaaacacagtctcagaagaagaaata

SEQ ID NO: 42 - protein, 36 aa, Bacillus licheniformis
MMGKGRIKVEERIKIETDAEMFKATLLDQTQSQKKK

SEQ ID NO: 43 - DNA, 231 bp, Bacillus licheniformis
atgaaagagaaaaaatcgtacgctgagctcatgaagtcccgcaatacccaaaaggtgaaagaacttgatgtaaccatcacggatatctacattcaaatggtccttgatgaatcgctttttaaacggcgtttgcacacgctgagcaagaagattaatgaagcattagacaaaggagataagcaatctttccttgagctttcaagagaatatacagcgctgaaaaagcacgca

SEQ ID NO: 44 - protein, 77 aa, Bacillus licheniformis
MKEKKSYAELMKSRNTQKVKELDVTITDIYIQMVLDESLFKRRLHTLSKKINEALDKGDKQSFLELSREYTALKKHA

SEQ ID NO: 45 - DNA, 627 bp, Bacillus licheniformis
gtgggaaaagaaaaaacaaaaaagccaatttataagaaatggtggttttggttaatcatcgttatcatcatcggggcagcagcatcaaatggtggaaattcagagcaagcttcatcaacaaataaagaaaaatccaccgagagtaaaacgactgaaacaaaacaagatacgaagaaagaagaaaaaaaggaagaaccgaaaaaagaggaaacaaaccctaaaatcggtgacgatgttaaagtcggtgatatgaattataaaatcactgggaagaaaacagcagatcaggtgggaccgtctgcattgcctcaaaaagctagcgataaataccttgttattgatgtcacattgaaaaataacggcaatgaaaaagtaacagtagacgcttctttcttcaagcttaaacgtggagaaaaaacctatgaagctgattctgctgcaagcatgtcagcgaaccaaagcgaggacggcaatattgacaataactttttccttcaaaacttgaatcctgattctaaaatcagtggaaaagtagtatttgatgtagctccggaagttgctaacgcaaaagacctacaattacaagtgcagactggtgcatggggaacggaaaccggaatcatcgat

SEQ ID NO: 46 - protein, 209 aa, Bacillus licheniformis
VGKEKTKKPIYKKWWFWLIIVIIIGAAASNGGNSEQASSTNKEKSTESKTTETKQDTKKEEKKEEPKKEETNPKIGDDVKVGDMNYKITGKKTADQVGPSALPQKASDKYLVIDVTLKNNGNEKVTVDASFFKLKRGEKTYEADSAASMSANQSEDGNIDNNFFLQNLNPDSKISGKVVFDVAPEVANAKDLQLQVQTGAWGTETGIID

SEQ ID NO: 47 - DNA, 1877 bp, Bacillus licheniformis
atgcaattagagatcgggaagcaatcgcagcaaaaccgtcacacgttgcaatttgaaaattggaggcagcacggggaattgatagctgcgcttttgtcgggtttgttgattcttgcaggctggctgttgtccggcaatgaaacattgtccgttgttctgtttattttagctttttgtatcggcggctttgctaaagcgaaagaaggtatacaagaaacgctgtcggaaaaaacgctgaatgttgaactcttgatgatttttgcggcggtcgggtctgcgctgatcggctactgggctgaaggggccgtgttaatttttatcttttctctcagcggagcgcttgaaacgtatacattaaataaaagcaaacgcgatttgacttcactgatgaaattggagccggaggaagccgttttgcttgaaaaagaaggaacaagaaccgtggcggcagccgatcttcaggcgggcgacctcattcttgtgaagcctggagaacgcattgcggcagacggagaaatcgaaaccggaaaaacgagtatcgacgaatcggctctaacgggcgaatccatcccagccgaaaaaacactcggagacgcggtttttgcgggtacggtcaatttgagcggatcgctcacggtccgtgtcacaaaggcaaatgaagattcgttgttcaaaaagatcattcggctcgttgagtctgcgcaaaacagcgtttcaccgtcgcaggcgttcattgagcgatttgaaaatatttacgttaaaggggttttgcttgctgtcggactgctgctctttctgccgcattttttgcttggctggagctggagcgagacattttacagagcgatggtgttcatggtcgtcgcttcgccgtgcgcccttgtcgcttcaatcatgcctgccgcgctgtcgctgatatcaaatggcgcaagaaacggcctgcttgtcaaaggcagcgtctttcttgaaaagcttggcaacagcaaaatcgttgcattggataaaacgggaacgattacgaacggaaagcccggcgtggaggatatgcttttagctgcagatatcgaggagcgcgaatgcttggaggctgctgctgcgattgagaagcagtcaggccatccgcttgccaaagcgattgtcgagtatgcagaagcaaaaggcatcaagccggccgcgaatgtgtcgattgaggagacgtcagggtttggcgttcaggctcgatacaatggagagacatggctgatcggcaaagccggatttgtcggggaagaggcagccgggcaatttctcacggcggctgttcaggagcttgccaagcagggaaaaacaattgtgttcatgaaaaaaggcgaaaaaatcgcggggtgttttgcattaaaagaccaaatcagaccggaagcaaaagcggtggtcgaagagctgaacgcgcttggcgttcagacggcgatgctgacaggggaccagcctgaaaccgcagcggccatcgcacgagaagcgggcttgaaaatcgtcgtttcagaatgccttcctgacagaaaagtagaggaagcgaaaaagctgaaaaaaacatacggaacaatcgttatggtgggagacggaatcaatgatgcaccggccctagccgccgctgatgtggggatcgcaatggggggaggaacagatgtcgcactggaaacggctgacgtcgttttaatgaaaaacgaattgacaggactgaccaaaatgattcggctctcccggaaaatgaatacgatcattaaacaaaacgtcattttctcgcttgctgtgatctgtcttttaatctgcagcaactttcttcaaattcttgatctgccgctcggtgtcatcgggcatgaaggcagcacgctgcttgtgat

SEQ ID NO: 48 - protein, 625 aa, Bacillus licheniformis
MQLEIGKQSQQNRHTLQFENWRQHGELIAALLSGLLILAGWLLSGNETLSVVLFILAFCIGGFAKAKEGIQETLSEKTLNVELLMIFAAVGSALIGYWAEGAVLIFIFSLSGALETYTLNKSKRDLTSLMKLEPEEAVLLEKEGTRTVAAADLQAGDLILVKPGERIAADGEIETGKTSIDESALTGESIPAEKTLGDAVFAGTVNLSGSLTVRVTKANEDSLFKKIIRLVESAQNSVSPSQAFIERFENIYVKGVLLAVGLLLFLPHFLLGWSWSETFYRAMVFMVVASPCALVASIMPAALSLISNGARNGLLVKGSVFLEKLGNSKIVALDKTGTITNGKPGVEDMLLAADIEERECLEAAAAIEKQSGHPLAKAIVEYAEAKGIKPAANVSIEETSGFGVQARYNGETWLIGKAGFVGEEAAGQFLTAAVQELAKQGKTIVFMKKGEKIAGCFALKDQIRPEAKAVVEELNALGVQTAMLTGDQPETAAAIAREAGLKIVVSECLPDRKVEEAKKLKKTYGTIVMVGDGINDAPALAAADVGIAMGGGTDVALETADVVLMKNELTGLTKMIRLSRKMNTIIKQNVIFSLAVICLLICSNFLQILDLPLGVIGHEGSTLLV

SEQ ID NO: 49 - DNA, 178 bp, Bacillus licheniformis
atggaacgcttttcagaagaagagagaaaactgttgctgaacgtacttttggaccatgagtatgccgtagagctactaagcagtgagatcaatgatatagaaactggtacaaaaaatgtggatagcctgacatataagaaactggttaccttatatgaccgtgtccggtctgaaaatt

SEQ ID NO: 50 - protein, 59 aa, Bacillus licheniformis
MERFSEEERKLLLNVLLDHEYAVELLSSEINDIETGTKNVDSLTYKKLVTLYDRVRSEN

SEQ ID NO: 51 - DNA, 537 bp, Bacillus licheniformis
atgattaatcagcttaaattgcgtccgcttgaaagagaagaccttccgtttgtccaccgtcttaacaacgatgcgaaaattatgtcatattggtttgaagaaccgtacgagacttttgttgagctgcaggatttatttgacaaacacattcacgaccaaagcgagcggcgctttatcatagagaaagagactgagatgatcggattggtagagctggtcgaaattgattatattcacaggcgggcggagtttcaaatcataattgatcccgagcatcaagggaacggttattcgtcaagcgcaacatatttggcaatgaactacgcattttccgtcttgaacttgcacaaattgtatttgatcgtcgacgaagataatgcaaaagcgattcacttgtataaaaaggcagggttcactatcgagagcgagctgcaggatgaatttttcgtcgacggctattatcgtaacgccattagaatgtgcatttttcaggatgagtttttatcacttaaaaaaagcaaagaggaaggcatgcag

SEQ ID NO: 52 - protein, 178 aa, Bacillus licheniformis
MINQLKLRPLEREDLPFVHRLNNDAKIMSYWFEEPYETFVELQDLFDKHIHDQSERRFIIEKETEMIGLVELVEIDYIHRRAEFQIIIDPEHQGNGYSSSATYLAMNYAFSVLNLHKLYLIVDEDNAKAIHLYKKAGFTIESELQDEFFVDGYYRNAIRMCIFQDEFLSLKKSKEEGM

SEQ ID NO: 53 - DNA, 207 bp, Bacillus licheniformis
atgcaccatatgaacgtatcatacttaagaaattgttttgccgagatgaaacagtatgagacagactgcatgaacaaactgatggatttcgctaagtttttgtatatccagggacatctgacattaaacgaatttcgcacaagtatgaaagttcttgaagcgaatggcgcacagcaccctgcttatgatatgaatacggacgccagc

SEQ ID NO: 54 - protein, 69 aa, Bacillus licheniformis
MHHMNVSYLRNCFAEMKQYETDCMNKLMDFAKFLYIQGHLTLNEFRTSMKVLEANGAQHPAYDMNTDAS

SEQ ID NO: 55 - protein, 69 aa, Bacillus licheniformis; identical to SEQ ID NO: 54

SEQ ID NO: 56 - protein, 160 aa, Bacillus licheniformis
MKKAILGFSLSAALLVPSSFAAAAGDGQLTSEQKELLEAKTEYVQSLPEQASVQSGVTAYAGKRLTIKRGSFLAWSKDYIDWYYNGKKVSKSSGSQDVGYVFPNVVRAKGIKRYYKSSGLHKWRAKKTLSFGTVTPWGDVELASSTFTDRRWVNKKGKYG

SEQ ID NO: 57 - DNA, 422 bp, Bacillus licheniformis
atgacaacaccgagtatggaagattacatagaacaaatttatatgctgattgaagaaaaaggatatgcaagagtctcagatatagccgaagctctggccgtccatccctcctcggttacaaaaatggttcaaaaactcgataaagacgaatatttgatttatgaaaagtatcgcggcctcgtgctgacgcctaaaggaaagaaaataggcaagcgtttagtatacagacatgaattattggagcagtttttacgaatcattggtgttgacgaagagaaaatttatgatgatgttgaaggaatcgaacatcatttaagctggaacagcattgaccgtatcggagatcttgtgcagtattttgaagacgacagcaaaagaatcgacgatttgagaagcgtccaaaaaagaaacgaacaggaaaa

SEQ ID NO: 58 - protein, 140 aa, Bacillus licheniformis
MTTPSMEDYIEQIYMLIEEKGYARVSDIAEALAVHPSSVTKMVQKLDKDEYLIYEKYRGLVLTPKGKKIGKRLVYRHELLEQFLRIIGVDEEKIYDDVEGIEHHLSWNSIDRIGDLVQYFEDDSKRIDDLRSVQKRNEQE

SEQ ID NO: 59 - DNA, 234 bp, Bacillus licheniformis
gtgccggacggttcaccatatcgtaaacgctatcaaccagccggtccggtgcggcagatgaaaaacaaacgtctgttcatactttcgttgattgtgttgagcgtggtcatgatcggagttcaggaaaccttcccaaacctgctgacgacagggttaatgactgtcgttattgcggcggcagtttttaatattttaaaagaatcgctgaataaaaaagatgaaacacacagcaaa

SEQ ID NO: 60 - protein, 78 aa, Bacillus licheniformis
MPDGSPYRKRYQPAGPVRQMKNKRLFILSLIVLSVVMIGVQETFPNLLTTGLMTVVIAAAVFNILKESLNKKDETHSK

SEQ ID NO: 61 - DNA, 210 bp, Bacillus licheniformis
atggctcaaaacaacagacaaagcagttctaaccaactattggttcctggtgctgctcaagctatcgaccaaatgaaattcgaaatcgcttctgaatttggcgttaaccttggagcagaaactacttctcgtgcaaacggttcagttggaggagaaatcactaagcgtttagtttctttcgctcaacagcaaatgggtggaacacaacaa

SEQ ID NO: 62 - protein, 70 aa, Bacillus licheniformis
MAQNNRQSSSNQLLVPGAAQAIDQMKFEIASEFGVNLGAETTSRANGSVGGEITKRLVSFAQQQMGGTQQ

SEQ ID NO: 63 - DNA, 1502 bp, Bacillus licheniformis
atgagcaacactgaacttgatttgctgaggcagcaggcgaatgaattaaacttgcaaatattaaagctgattaacgagcgaggaagaatcgttcaggagattggaaaagcgaaggaagcacaaggcatcaaccgctacgatcctgtcagagaaagagcgatgctgaacgaaattattgaaaataacgacggaccgtttgaaaactcgacgatccagcatatcttcaaagagattttcaaagccgggcttgaactgcaggaagacgatcacagcaaagcgctgctcgtttcccgcaagaaaaagcctgaaaatacaatcgttgatctgaaaggcgaaaaaatcggcgacggagaacaaagatttatcgtcggtccgtgtgcggttgaaagctacgaacaagtagcggaagtcgcagcggcagctaaaaagcaaggcttgaaactgcttcgcggcggagctttcaaaccgcgtacaagcccgtacgacttccaaggcctcggcgtggaaggcctgcaaatcttaaagcgtgttgctgatgagtatgatctggccgtcatcagtgagatcgtgaatccgcagcatattgaagaagccattgattacatcgatgtcatccaaatcggcgcccgcaacatgcagaacttcgagctcttaaaagcggccggttcagtgaagaagccggttctgctgaagcgcggacttgccgcaacgctgaaggaattcatcaatgcagcggagtacatcatgtcgcagggcaatgatcaaatcatcctttgtgaacgcggaatcagaacgtatgaaacagcgactagaaatacgcttgatatctcagctgtgccgatcctgaagcaggaaactcaccttcctgtattcgtggatgtcactcattcaaccggacgccgcgacctgcttcttccgacagcaaaagcagcgcttgcgatcggagctgacggtgtcatggccgaggtccatcctgatccttctgtcgcgctttccgactcagctcagcaaatggatatcccgacatttgaaaaatggttaaatgaactgaagccgctcgttcaagtaaaagcataattgaacactgaattaaagtacatgcttcaatccgttctaaaagaagaattgagtccgatcaatcagcgccttgatggaatcgacaagcgcttagacaaaatcgacgcacgcttcgttgagatagacaagcgcttcgatgaagtggacgcacgcttcgttgaagtagataagcgctttaacgcaatcgacaagcgcttcaaagaaatagacgggcgcttaaacaaagtagaaaaccgcttaaacgcaatggacaagcggctgaatcggcttgaaacagatatagatgaactgaaaagagggcaggagaggctcccgaaaacgatcatcgagaacatcggacaatttacggagaacattgtcgaacatgccgatgataaggcggctgccttgaatgacagggtttttagcgtcgaaaccgcaataca

SEQ ID NO: 64 - protein, 147 aa, Bacillus licheniformis
MNTELKYMLQSVLKEELSPINQRLDGIDKRLDKIDARFVEIDKRFDEVDARFVEVDKRFNAIDKRFKEIDGRLNKVENRLNAMDKRLNRLETDIDELKRGQERLPKTIIENIGQFTENIVEHADDKAAALNDRVFSVETAIQRIYRL

SEQ ID NO: 65 - DNA, 375 bp, Bacillus licheniformis
atgaaactaaattatgattgtgtccgctcaattcttctagaattagaggaaaatttaactcttaacgatggcgtcactttatatcagctcaaagattttgagacattcaaagagtatggctatgaaacttccgtttacgctttaaccaagttaatcgaagctgactttttaaacggttcggtttcgcgcgcagacaataagattgactatattggtgttggctctattacttgggatggacatcaatttttagacaacattcgtgacaatgctgtttggtctaaaacgaaagatgccgttaagtcgttatcaagcgtttccttgtccatactttcaaatgtcggagaaagcatcacgaaaaagcttatcggttta

SEQ ID NO: 66 - protein, 124 aa, Bacillus licheniformis
MKLNYDCVRSILLELEENLTLNDGVTLYQLKDFETFKEYGYETSVYALTKLIEADFLNGSVSRADNKIDYIGVGSITWDGHQFLDNIRDNAVWSKTKDAVKSLSSVSLSILSNVGESITKKLIG

SEQ ID NO: 67 - DNA, 458 bp, Bacillus licheniformis
atgatctctcaacaattaaaacagcaaaatcctgtacttgaaaactcaatgaatacgaatttgtcaaactggttcatcctttacacgaagcttcaccgttttcactggtacgtaaaagggccgcagttctttaccctacatgaaaaatttgaagagctatacaaccatgcgtcagaaacagcagatgtgatcgcggaacgcttgctggccatcggcggacagccgctcgccacaatgaaagaatacattgaccacggcacaattgaggaaaacggagccgaaaaaacggccgaagaaatggtttccgcactggtaagcgattaccgtcaaatccgcgatgaaattcagcataccatcgaacttgcggaagataaatcagatcattctaccgctgacctttatatcgccctgacagaggaaattgataagcagatttggatgctttcttcatttttgga

SEQ ID NO: 68 - protein, 152 aa, Bacillus licheniformis
MISQQLKQQNPVLENSMNTNLSNWFILYTKLHRFHWYVKGPQFFTLHEKFEELYNHASETADVIAERLLAIGGQPLATMKEYIDHGTIEENGAEKTAEEMVSALVSDYRQIRDEIQHTIELAEDKSDHSTADLYIALTEEIDKQIWMLSSFL

SEQ ID NO: 69 - DNA, 373 bp, Bacillus licheniformis
atgaatgagaagattttaatcgtagacgaccagtacgggattcgggttctgctgaatgaagttttcaataaagaagggtacaaaaccttccaggccgcaaacgggattcaagcgcttgacattgtgaaaaaccagcgccccgacctcgttctgctcgatatgaaaatccccggaatggacggaattgaaattttaaaaagaatgaagatcatagacgaggggatccgcgtcatcatcatgacggcctacggagagctcgacatgatccaggaatcgaaggagctcggagccctgacacactttgctaagccttttgacatcgacgaaatccgcgatgccgtcaaaacgtatctgcccataaagtccaacggat

SEQ ID NO: 70 - protein, 122 aa, Bacillus licheniformis
MNEKILIVDDQYGIRVLLNEVFNKEGYKTFQAANGIQALDIVKNQRPDLVLLDMKIPGMDGIEILKRMKIIDEGIRVIIMTAYGELDMIQESKELGALTHFAKPFDIDEIRDAVKTYLPIKS

SEQ ID NO: 71 - DNA, 523 bp, Bacillus licheniformis
ttgcttaaaattttcaccactcaattgacgggaatcttcaaccggattcaagagggcgaggcccaatcgatagaggacggcgcccgcttgttggctcaggcggtcatcagtgatcattcggtttatgtatacggaaaaaatgaattggaaggcattttgaaagaagcgatgtacagttctgaaccgttcccctcagtcaaaccgctgcagaaggacgaagaaaactggcccgattttgaaatgacggacaaagtgctgatgttctgcgccggttcagcggatgacgaagaactgaaaatggcggaaaaactgtatgaaaaaggaatcggacttgttgtcgtctccccttcgggaaaagacggcgtcccgatcgcatccttcgccgatgtccatatcgattcaaagctgagaatgccgcttcttcccgatgaagacggaacaaggtacggatttccgtccctgatggtcagcctctatatttatcatgccctatcctttacattaaaggaaatcctccaggaat

SEQ ID NO: 72 - protein, 174 aa, Bacillus licheniformis
MLKIFTTQLTGIFNRIQEGEAQSIEDGARLLAQAVISDHSVYVYGKNELEGILKEAMYSSEPFPSVKPLQKDEENWPDFEMTDKVLMFCAGSADDEELKMAEKLYEKGIGLVVVSPSGKDGVPIASFADVHIDSKLRMPLLPDEDGTRYGFPSLMVSLYIYHALSFTLKEILQE

SEQ ID NO: 73 - DNA, 266 bp, Bacillus licheniformis
atgagcaaaacgattaaacttaaccatgcagcggttatgaagaagctggaacaagtaagcagcacgcttcaagccgtatctttaaaaagcccgccagccggagcgctcgggcggaacaaccttgattttacgaaaaagtggcttgaacgagaagccgaaatttgcaatatggtcaaacagtataaagaggctgttcgtaaaaacattgaggacacccgctcaaatgtggacacgctgaaggaacaggatgaggcgattgcccgaag

SEQ ID NO: 74 - protein, 88 aa, Bacillus licheniformis
MSKTIKLNHAAVMKKLEQVSSTLQAVSLKSPPAGALGRNNLDFTKKWLEREAEICNMVKQYKEAVRKNIEDTRSNVDTLKEQDEAIAR

SEQ ID NO: 75 - DNA, 1396 bp, Bacillus licheniformis
atgaaatataaaacattagctcaatttccgaaagattttttgtggggcgcgtctacttccgcttatcaagtggaaggcgcttgggacgaagatggaaaagggccttctgtcatcgatgcgcgcgaaagctacccggaagggacaaccgattttaaagtcgcaagcgaccattaccagcgctataaagaagatatcgctttatttgcggaaatgggcttcaaagcgtaccgtttttcgattgcctggacgcgcatcattccggacggggacggtgatattaatccgaagggaatcgaattttacagccgtttgatcgatgaacttctaaagtatggaatcgaaccaattgttacgatgtaccactttgatctgccgaatgctttgcagaaaaaaggcggctggtcggacagggccacgattgatgcttttgaaaagtatgcgaaggtcctttttgaaagctacggtgaccgcgtcaaatactggctgaccatcaatgagcaaaatatgatgatcctccacggatctgcactcggtacactcgatccgaacttggaaaatccgaaaaaagagctttatcagcaaaaccatcacatgctcgtcgcacaggcgaaagcgatcaagctttgccatgagatgctgccggaagcaaaaatcggtcctgcgccgaatattgcgctcatctatcccgcttcttcgaaaccggaggacgtgctggcggcttttaactataatgcgatccgaaactggctttacttggatatggccgtattcggacggtacaatacaacagcgtgggcatatatgaaagaaaaaggctgcacaccggtcatcgctgaaggggatatggacattctgcggtcggccaagccggattttatcgcgtttaactactatacatcgcaaacggctgaagcaagcaggggtgatggcagcgacacggctgctcgaggcggagaccagcatttgcagacgggagaagaaggcgtatataggggaagcagcaatccgcacctaaagaaaaacgcatttggctgggagatcgaccctgtcggtttccgttcgacgctgcgcgaaatttacgaccgctaccagctgccgctgatcgtcactgagaacggcctcggcgcgtttgatcagcttgaagacggagatgtcgtaaatgacgattaccgcatcgattatttaaaagagcatatcaagcaaattcagctggcaatcacggatggagtcgatgttttcggctactccccatggtctgccatcgacttaatttcgacccatcaaggctgttcaaaacgctacggatttatttatgtgaaccgcgatgaatttgatttgaaagacttgcgccgcattcgcaaaaaaagcttttactggtataaaaacctgattgcta

SEQ ID NO: 76 - protein, 465 aa, Bacillus licheniformis
MKYKTLAQFPKDFLWGASTSAYQVEGAWDEDGKGPSVIDARESYPEGTTDFKVASDHYQRYKEDIALFAEMGFKAYRFSIAWTRIIPDGDGDINPKGIEFYSRLIDELLKYGIEPIVTMYHFDLPNALQKKGGWSDRATIDAFEKYAKVLFESYGDRVKYWLTINEQNMMILHGSALGTLDPNLENPKKELYQQNHHMLVAQAKAIKLCHEMLPEAKIGPAPNIALIYPASSKPEDVLAAFNYNAIRNWLYLDMAVFGRYNTTAWAYMKEKGCTPVIAEGDMDILRSAKPDFIAFNYYTSQTAEASRGDGSDTAARGGDQHLQTGEEGVYRGSSNPHLKKNAFGWEIDPVGFRSTLREIYDRYQLPLIVTENGLGAFDQLEDGDVVNDDYRIDYLKEHIKQIQLAITDGVDVFGYSPWSAIDLISTHQGCSKRYGFIYVNRDEFDLKDLRRIRKKSFYWYKNLIA

SEQ ID NO: 77 - DNA, 1830 bp, Bacillus licheniformis
atgaatgttcaatcaatggcaaaagaaattctggcgcgcgtcggcggggagaagaacgttgtatcgctagtccattgcgcgacaaggctccgcttcaaactgaaagaccgttccaaagcagacagagaagcgcttgaaaatacggatggcgtggtaaccgtggtggagagcggcgggcaatttcaagtcgttatcggcaataacgttcctgaagtatataaagaaatcggccggatctctcaactgttggaaagttctgcggccgatcacagtcaaaaagagaaaggaagcctcgccggtagattagtagatgtcgtatccagcattttcactccgctgctcggcgtcatggcgggagcggggattttaaaaggcctgcttttgatttgcacaaacgccggctggctctcgccggaagagacgacatatacgattctatacgcggcagccgacagcctgttttatttcctgcctttgctgctcgccgttacggccgccaaaaaattcggagcgaacccgttcatagcgctgacgattgccggagcgctgatctatccgacgatactcgaactgaaaaacagcggcgcccatacggagtttttcggcattccggtcgtcttgatgaattatacgtcgaccgttatcccgattatccttgcggtatttgtgatgagctatcttgaaagattatgtatgcgctttattcatgaaagcgtgaagaactttatcacccctttattatgcctgacggtgatggtgccgttaactttgatcgtattcggaccgctcggcgtttacacaggaaacgggatcgcggcggcgattctgtccgtttttgatttcagcccgattctggcaggagcgattattgcggccttatggcaaatccttgtcatcttcgggattcactgggggatcgtccctgtcattttgaacaacattgccgtccacggcaaggactacattaagccggcgacggcagccgccgtgtttgcccaaacaggagccgcatttggcgtcatgctgaagacgaaaaacaagaagctgaaagcattggcaggatcagctgccgttaccgggatattcgggattacagagccggccgtctacggggtgacgctcaggctgaaaaagccgtttgtatgcggtgtcatcagcgcggcggcaggcggagccattatcggatactccggcagcgtcgccctcgcttccggcgctccgggcttgttgacgattccgattttttacggaccgggctttctcggcttcatcatcggcatttcagtttcatttgttttatcgattttgctcacttacattgtcggctttgacgaccctgtggaggtgacaaaagaggagcctgttgaaaaaagcgccggtgaaccgatttacagccctttgcaaggagaagtcctgccgttaacagaagtatcagataaagtgttcgcatcgggggcgcttggagagggaatcgcggtggttccgtcaaaaggcgttgtcaccgcccctgcggacggcatcgtgacaacggcatttccgacgggtcacgcatacggcataacgaccgaaagcggagccgagattttgattcatattggaatggacacagtcaggctcgaaggaaagcacttcaatcctaaagccgtgcaggggcaaaatgtgaaacggggtgatatactcgcagaattcgatctggacgctttgaaagaagaagggtttgacgtgaaaacgccgatcatcgttacaaattccggtcaatacacggatgtcattccaacggatcaaaaaaaggtgaaaactgaagaacggatcatcactttaatttcatca

SEQ ID NO: 78 - protein, 609 aa, Bacillus licheniformis
MNVQSMAKEILARVGGEKNVVSLVHCATRLRFKLKDRSKADREALENTDGVVTVVESGGQFQVVIGNNVPEVYKEIGRISQLLESSAADHSQKEKGSLAGRLVDVVSSIFTPLLGVMAGAGILKGLLLICTNAGWLSPEETTYTILYAAADSLFYFLPLLLAVTAAKKFGANPFIALTIAGALIYPTILELKNSGAHTEFFGIPVVLMNYTSTVIPIILAVFVMSYLERLCMRFIHESVKNFITPLLCLTVMVPLTLIVFGPLGVYTGNGIAAAILSVFDFSPILAGAIIAALWQILVIFGIHWGIVPVILNNIAVHGKDYIKPATAAAVFAQTGAAFGVMLKTKNKKLKALAGSAAVTGIFGITEPAVYGVTLRLKKPFVCGVISAAAGGAIIGYSGSVALASGAPGLLTIPIFYGPGFLGFIIGISVSFVLSILLTYIVGFDDPVEVTKEEPVEKSAGEPIYSPLQGEVLPLTEVSDKVFASGALGEGIAVVPSKGVVTAPADGIVTTAFPTGHAYGITTESGAEILIHIGMDTVRLEGKHFNPKAVQGQNVKRGDILAEFDLDALKEEGFDVKTPIIVTNSGQYTDVIPTDQKKVKTEERIITLIS

SEQ ID NO: 79 - DNA, 821 bp, Bacillus licheniformis
gtgaaaattgccaaagtgatcaacaacaatgtgatcagtgttttaaatgaacagggtcaggaattagtggtcatgggcaggggaatcgcttttcaaaaaaagcctggcgaagcggtggatgaatcgagaatcgagaagattttcaggcttgataataaagatgtatcagaaaggtttaagacgctgttggacgaaattccaattgaatttatggaaatgtctgaagaaattatctcctatgcgaaattaaagctcggcaaaaagctgaatgacagcatttatgtctcgctgaccgaccatattcatttcgccgtcgaacggcataaaaagggactggatattaaaaatgccctgctttgggagacgaaacggctgtataaagatgagttcgccatcggcaaagaggcgctggccatcattgaaaagaagacggggacagctcttccggaggatgaagccgcctttatcgcgctccatatcgtaaacgccgagctgaatgaagaaatgccgaacatcgtcaatattacgaaagtcatgcaggagattttaagcatcgtcaagtatcactttcatatcgaatttgacgaagaatcgcttcactattaccgcttcattacccatttgaaatttttcgcccagcggctgttcagcggaacctatatggaaagccgggacgactttttatttgaaaccgtcaaaaataagtaccgggacgcttatgtttgtacaaataaaatcaggcagtatatcgaaaaagaatacggtcatcagctgacaaacgaagagcttctgtatttgacgattcatatcgagcgagtcgt

SEQ ID NO: 80 - protein, 273 aa, Bacillus licheniformis
MKIAKVINNNVISVLNEQGQELVVMGRGIAFQKKPGEAVDESRIEKIFRLDNKDVSERFKTLLDEIPIEFMEMSEEIISYAKLKLGKKLNDSIYVSLTDHIHFAVERHKKGLDIKNALLWETKRLYKDEFAIGKEALAIIEKKTGTALPEDEAAFIALHIVNAELNEEMPNIVNITKVMQEILSIVKYHFHIEFDEESLHYYRFITHLKFFAQRLFSGTYMESRDDFLFETVKNKYRDAYVCTNKIRQYIEKEYGHQLTNEELLYLTIHIERV

SEQ ID NO: 81 - DNA, 1387 bp, Bacillus licheniformis
atgactgaacaaacgaaaaagtttcctgaaggttttttatggggcggagcggttgccgcaaaccaagtggaaggcgcctataatgtcggcgggaaaggactctcgacagccgatgtgtcgccgaacggcgtcatgtatccattcgatgagtcgatggagtcattgaacctgtatcatgaaggcatcgatttttaccaccgctacaaagaagatatcgctcttttcgccgaaatgggatttaaagcattccggacatcgattgcctggacgcggatttttcctaacggcgatgaaactgaaccgaatgaagagggactcgaattttatgatcgcctctttgacgagctattaaaatacaatattgagccagtggtgacgatttcccactacgaaatgccgctcggtctgattaaaaaatacggcggctggaaaaaccggaaagtgatcgattgctatgagcattatgcgaaaacggttttcacccgctataaagaaaaagtaaaatactggatgacattcaatgaaatcaacatggttctgcatgcgccgtttacaggcggaggccttgtgtttgaagaaggcgaaaacaagttaaatgcgatgtaccaagcggcgcatcatctatttgtcgcaagcgctcttgccgttaaagcggggcacgacatcattccggacgctaaaatcggctgcatgatcgccgcaacgacgacatacccgatgacgccaaagccggaagacgtgctcgctgcgatggagaatgagagaagaacgctgtttttctcggatgtacaggcgcgcggggcttatccgggctatatgaagcgcttctttaaggaaaacggaattacgattgaaatggctgaaggtgatgaagacatcttaaaggaaaacaccgtcgactatatcggtttcagctactacatgtcaatggtcgcaagcacgagtccggaagacttggcaaaaacggaaggcaacctgctcggcggcgtcaaaaatccgtaccttgaatcgtccgaatggggctggcagatcgatcctaaagggatccgcattacgctgaatacattgtacgaccgctatcaaaagccgcttttcattgttgaaaacgggctcggcgccgtcgatgtcgtcgaagaagacggctccatccaggatgactacagaatcaactatttgcgcgatcatttaaaagaagtaagagaagccattgcagacggcgtcgacttaatcggctacacatcatggggcccgatcgacctggtcagcgcatccaccgccgaaatgaaaaagcgctacggctatatttacgtcgatcgtgacaatgaaggaaaaggcacgctttcaagaacgagaaagaaaagcttttactggtataagaaagtaatcg

SEQ ID NO: 82 - protein, 462 aa, Bacillus licheniformis
MTEQTKKFPEGFLWGGAVAANQVEGAYNVGGKGLSTADVSPNGVMYPFDESMESLNLYHEGIDFYHRYKEDIALFAEMGFKAFRTSIAWTRIFPNGDETEPNEEGLEFYDRLFDELLKYNIEPVVTISHYEMPLGLIKKYGGWKNRKVIDCYEHYAKTVFTRYKEKVKYWMTFNEINMVLHAPFTGGGLVFEEGENKLNAMYQAAHHLFVASALAVKAGHDIIPDAKIGCMIAATTTYPMTPKPEDVLAAMENERRTLFFSDVQARGAYPGYMKRFFKENGITIEMAEGDEDILKENTVDYIGFSYYMSMVASTSPEDLAKTEGNLLGGVKNPYLESSEWGWQIDPKGIRITLNTLYDRYQKPLFIVENGLGAVDVVEEDGSIQDDYRINYLRDHLKEVREAIADGVDLIGYTSWGPIDLVSASTAEMKKRYGYIYVDRDNEGKGTLSRTRKKSFYWYKKVI

SEQ ID NO: 83 - DNA, 1820 bp, Bacillus licheniformis
atggattataataaagtatcgaaggacattttacaactcgtgggcggtgaagagaacgtacagagcgtgattcactgcatgacaagactgcgtttcaatctttatgacaatgcgaaggcagaccgcgcgaaactggaaagtcttccggctgtaatgggcaccaacatcagcggccagcagtttcaaatcatcattggaaatgatgtccctaaggtgtataaagcgatcattgccaacagcgggctcagcgatgaaaaagcgggcgagcagcaagctggcaaaaagaaaaacgtgctgtccgccatttttgatgtgatatcaggcgtatttacgccgattctcccggcgatcgccggagcgggtatgatcaaggggatcattgcaatcgccgtcacgttcggctggatgagcgaaactagccaggtccacaccattttatccgccatcggcgacggagcattttacttcctgccgattttgctggcggtcagtgccgcgagaaaattcggcagtaatccttatgttgcggcggcgatcggagcggcgattctgcatcccgatctgacagcgcttctcggttcagggaaaagcatttcctttgtcggattgcctgtaaccgctgccacttattcgtcgaccgtcattccgatcctgctcgcgatttggattgcatcttacgttgagaaatggattgacaaagtcaccccgacttcgttgaagatgatttttgtaccgacgctgacgctgctggttgtcgtgcctgtcacattaattacggtcggtccgctcggtgcgattgcagggaactatctgtcaatcggtgtgaacggtttatttgaaaatgccggtttaatcacgatgatccttttagcaggaacgttctcgctgatcgtcatgacaggaatgcactatgctttcattccggttatgttcaacaacattacgcaaaacggctacgattacttgatacctgcgatgttcttggcgaatatggggcaggctggcgcgtcatttgccgtcttcctgcgatccagaaataagaaattcaaatcattgtcgctgacgacaagcatcacggctttgatggggattacagagccggcgatgtacggtgtcaacatgaggctgaaaaagccgtttgtatccgcgcttctcggcgccgctgtcggaggagcattttacggcatcaccggcgtagcagcatatattattggcggaaacgtcggtttgccgggaattacgacgtttatcggcccgacttttatacaggcaatgatcggtatcgtcatcgcgttctttgccgcaacggcgtttgcttttgtattggggtttgaagacattccttcagatgaagccgctgaacaaggagccgctccatctgaagcgggcgcgggagagatcattcaaagcccgctgaaaggcgaagtcaaagcattgagtgaagtggatgatgcgacattttctggagaagtcatgggaaaaggcgtcgccattgagcctgaagaaggcaaagtggtgtcgccggtatcaggcacgatcacaaccgtttttcaaacgaagcacgccctcggcattacaagcgacaatggggcggaaattattatccatatcggaatcgacacggtgaaattgaacggcgagcactttaccgtgcatgtcaataaaggcgacgctgtaaaaccgggagacgagcttgtctcatttgatatggatgcgattaaggatgcaggctatcagttgatcacgccggttatcatcacaaatacggaccggtaccagtcgatcaaacctttgaaatcagatgaaagcgttgacattga

SEQ ID NO: 84 - protein, 604 aa, Bacillus licheniformis
MDYNKVSKDILQLVGGEENVQSVIHCMTRLRFNLYDNAKADRAKLESLPAVMGTNISGQQFQIIIGNDVPKVYKAIIANSGLSDEKAGEQQAGKKKNVLSAIFDVISGVFTPILPAIAGAGMIKGIIAIAVTFGWMSETSQVHTILSAIGDGAFYFLPILLAVSAARKFGSNPYVAAAIGAAILHPDLTALLGSGKSISFVGLPVTAATYSSTVIPILLAIWIASYVEKWIDKVTPTSLKMIFVPTLTLLVVVPVTLITVGPLGAIAGNYLSIGVNGLFENAGLITMILLAGTFSLIVMTGMHYAFIPVMFNNITQNGYDYLIPAMFLANMGQAGASFAVFLRSRNKKFKSLSLTTSITALMGITEPAMYGVNMRLKKPFVSALLGAAVGGAFYGITGVAAYIIGGNVGLPGITTFIGPTFIQAMIGIVIAFFAATAFAFVLGFEDIPSDEAAEQGAAPSEAGAGEIIQSPLKGEVKALSEVDDATFSGEVMGKGVAIEPEEGKVVSPVSGTITTVFQTKHALGITSDNGAEIIIHIGIDTVKLNGEHFTVHVNKGDAVKPGDELVSFDMDAIKDAGYQLITPVIITNTDRYQSIKPLKSDESV

SEQ ID NO: 85 - DNA, 570 bp, Bacillus licheniformis
atgagcacagaggatatgacaaaggatacgtatgaagtaaacagttcgacaatggctgtcctgcctctgggagagggggagaaacccgcctcaaaaatacttgagaccgacaggactttccgcgtcaatatgaagccgtttcaaattatcgaaagaagctgccgctatttcggatcgagctatgcgggaagaaaagcgggcacatatgaagtcattaaagtttcccataaaccgccgatcatggtggatcactcaaacaacatttttcttttccccacattttcctcaactcgtcctcagtgcgggtggctttcccatgcgcatgttcacgagttttgcgcggcaaagtatgacaacacgtttgtcacgtttgtcaacggggaaacgctggagctgcccgtatccatctcatctttcgaaaaccaggtttaccgaacggcatggctgagaacaaaatttatcgacaggattgaaggaaaccccatgcagaagaaacaggaatttatgctctatccgaaagaagaccggaatcagctgatatacgaattcatcctcagggagctgaaaaag

SEQ ID NO: 86 - protein, 189 aa, Bacillus licheniformis
MSTEDMTKDTYEVNSSTMAVLPLGEGEKPASKILETDRTFRVNMKPFQIIERSCRYFGSSYAGRKAGTYEVIKVSHKPPIMVDHSNNIFLFPTFSSTRPQCGWLSHAHVHEFCAAKYDNTFVTFVNGETLELPVSISSFENQVYRTAWLRTKFIDRIEGNPMQKKQEFMLYPKEDRNQLIYEFILRELK

SEQ ID NO: 87 - DNA, 36 bp, Bacillus licheniformis
gccgcagccatttccagagccgcagccatttccaga

SEQ ID NO: 88 - protein, 1368 aa, Streptococcus pyogenes [sequence omitted]

SEQ ID NO: 89 - protein, 1307 aa, Acidomiococcus sp.
MTQFEGFTNLYQVSKTLRFELIPQGKTLKHIQEQGFIEEDKARNDHYKELKPIIDRIYKTYADQCLQLVQLDWENLSAAIDSYRKEKTEETRNALIEEQATYRNAIHDYFIGRTDNLTDAINKRHAEIYKGLFKAELFNGKVLKQLGTVTTTEHENALLRSFDKFTTYFSGFYENRKNVFSAEDISTAIPHRIVQDNFPKFKENCHIFTRLITAVPSLREHFENVKKAIGIFVSTSIEEVFSFPFYNQLLTQTQIDLYNQLLGGISREAGTEKIKGLNEVLNLAIQKNDETAHIIASLPHRFIPLFKQILSDRNTLSFILEEFKSDEEVIQSFCKYKTLLRNENVLETAEALFNELNSIDLTHIFISHKKLETISSALCDHWDTLRNALYERRISELTGKITKSAKEKVQRSLKHEDINLQEIISAAGKELSEAFKQKTSEILSHAHAALDQPLPTTLKKQEEKEILKSQLDSLLGLYHLLDWFAVDESNEVDPEFSARLTGIKLEMEPSLSFYNKARNYATKKPYSVEKFKLNFQMPTLASGWDVNKEKNNGAILFVKNGLYYLGIMPKQKGRYKALSFEPTEKTSEGFDKMYYDYFPDAAKMIPKCSTQLKAVTAHFQTHTTPILLSNNFIEPLEITKEIYDLNNPEKEPKKFQTAYAKKTGDQKGYREALCKWIDFTRDFLSKYTKTTSIDLSSLRPSSQYKDLGEYYAELNPLLYHISFQRIAEKEIMDAVETGKLYLFQIYNKDFAKGHHGKPNLHTLYWTGLFSPENLAKTSIKLNGQAELFYRPKSRMKRMAHRLGEKMLNKKLKDQKTPIPDTLYQELYDYVNHRLSHDLSDEARALLPNVITKEVSHEIIKDRRFTSDKFFFHVPITLNYQAANSPSKFNQRVNAYLKEHPETPIIGIDRGERNLIYITVIDSTGKILEQRSLNTIQQFDYQKKLDNREKERVAARQAWSVVGTIKDLKQGYLSQVIHEIVDLMIHYQAVVVLENLNFGFKSKRTGIAEKAVYQQFEKMLIDKLNCLVLKDYPAEKVGGVLNPYQLTDQFTSFAKMGTQSGFLFYVPAPYTSKIDPLTGFVDPFVWKTIKNHESRKHFLEGFDFLHYDVKTGDFILHFKMNRNLSFQRGLPGFMPAWDIVFEKNETQFDAKGTPFIAGKRIVPVIENHRFTGRYRDLYPANELIALLEEKGIVFRDGSNILPKLLENDDSHAIDTMVALIRSVLQMRNSNAATGEDYINSPVRDLNGVCFDSRFQNPEWPMDADANGAYHIALKGQLLLNHLKESKDLKLQNGISNQDWLAYIQELRN

SEQ ID NO: 90 - protein, 887 aa, N. gregoryi
MTVIDLDSTTTADELTSGHTYDISVTLTGVYDNTDEQHPRMSLAFEQDNGERRYITLWKNTTPKDVFTYDYATGSTYIFTNIDYEVKDGYENLTATYQTTVENATAQEVGTTDEDETFAGGEPLDHHLDDALNETPDDAETESDSGHVMTSFASRDQLPEWTLHTYTLTATDGAKTDTEYARRTLAYTVRQELYTDHDAAPVATDGLMLLTPEPLGETPLDLDCGVRVEADETRTLDYTTAKDRLLARELVEEGLKRSLWDDYLVRGIDEVLSKEPVLTCDEFDLHERYDLSVEVGHSGRAYLHINFRHRFVPKLTLADIDDDNIYPGLRVKTTYRPRRGHIVWGLRDECATDSLNTLGNQSVVAYHRNNQTPINTDLLDAIEAADRRVVETRRQGHGDDAVSFPQELLAVEPNTHQIKQFASDGFHQQARSKTRLSASRCSEKAQAFAERLDPVRLNGSTVEFSSEFFTGNNEQQLRLLYENGESVLTFRDGARGAHPDETFSKGIVNPPESFEVAVVLPEQQADTCKAQWDTMADLLNQAGAPPTRSETVQYDAFSSPESISLNVAGAIDPSEVDAAFVVLPPDQEGFADLASPTETYDELKKALANMGIYSQMAYFDRFRDAKIFYTRNVALGLLAAAGGVAFTTEHAMPGDADMFIGIDVSRSYPEDGASGQINIAATATAVYKDGTILGHSSTRPQLGEKLQSTDVRDIMKNAILGYQQVTGESPTHIVIHRDGFMNEDLDPATEFLNEQGVEYDIVEIRKQPQTRLLAVSDVQYDTPVKSIAAINQNEPRATVATFGAPEYLATRDGGGLPRPIQIERVAGETDIETLTRQVYLLSQSHIQVHNSTARLPITTAYADQASTHATKGYLVQTGAFESNVGFL

SEQ ID NO: 91 - DNA, 12203 bp, Streptococcus pyogenes
atggataagaaatactcaataggcttagatatcggcacaaatagcgtcggatgggcggtgatcactgatgaatataaggttccgtctaaaaagttcaaggttctgggaaatacagaccgccacagtatcaaaaaaaatcttataggggctcttttatttgacagtggagagacagcggaagcgactcgtctcaaacggacagctcgtagaaggtatacacgtcggaagaatcgtatttgttatctacaggagattttttcaaatgagatggcgaaagtagatgatagtttctttcatcgacttgaagagtcttttttggtggaagaagacaagaagcatgaacgtcatcctatttttggaaatatagtagatgaagttgcttatcatgagaaatatccaactatctatcatctgcgaaaaaaattggtagattctactgataaagcggatttgcgcttaatctatttggccttagcgcatatgattaagtttcgtggtcattttttgattgagggagatttaaatcctgataatagtgatgtggacaaactatttatccagttggtacaaacctacaatcaattatttgaagaaaaccctattaacgcaagtggagtagatgctaaagcgattctttctgcacgattgagtaaatcaagacgattagaaaatctcattgctcagctccccggtgagaagaaaaatggcttatttgggaatctcattgctttgtcattgggtttgacccctaattttaaatcaaattttgatttggcagaagatgctaaattacagctttcaaaagatacttacgatgatgatttagataatttattggcgcaaattggagatcaatatgctgatttgtttttggcagctaagaatttatcagatgctattttactttcagatatcctaagagtaaatactgaaataactaaggctcccctatcagcttcaatgattaaacgctacgatgaacatcatcaagacttgactcttttaaaagctttagttcgacaacaacttccagaaaagtataaagaaatcttttttgatcaatcaaaaaacggatatgcaggttatattgatgggggagctagccaagaagaattttataaatttatcaaaccaattttagaaaaaatggatggtactgaggaattattggtgaaactaaatcgtgaagatttgctgcgcaagcaacggacctttgacaacggctctattccccatcaaattcacttgggtgagctgcatgctattttgagaagacaagaagacttttatccatttttaaaagacaatcgtgagaagattgaaaaaatcttgacttttcgaattccttattatgttggtccattggcgcgtggcaatagtcgttttgcatggatgactcggaagtctgaagaaacaattaccccatggaattttgaagaagttgtcgataaaggtgcttcagctcaatcatttattgaacgcatgacaaactttgataaaaatcttccaaatgaaaaagtactaccaaaacatagtttgctttatgagtattttacggtttataacgaattgacaaaggtcaaatatgttactgaaggaatgcgaaaaccagcatttctttcaggtgaacagaagaaagccattgttgatttactcttcaaaacaaatcgaaaagtaaccgttaagcaattaaaagaagattatttcaaaaaaatagaatgttttgatagtgttgaaatttcaggagttgaagatagatttaatgcttcattaggtacctaccatgatttgctaaaaattattaaagataaagattttttggataatgaagaaaatgaagatatcttagaggatattgttttaacattgaccttatttgaagatagggagatgattgaggaaagacttaaaacatatgctcacctctttgatgataaggtgatgaaacagcttaaacgtcgccgttatactggttggggacgtttgtctcgaaaattgattaatggtattagggataagcaatctggcaaaacaatattagattttttgaaatcagatggttttgccaatcgcaattttatgcagctgatccatgatgatagtttgacatttaaagaagacattcaaaaagcacaagtgtctggacaaggcgatagtttacatgaacatattgcaaatttagctggtagccctgctattaaaaaaggtattttacagactgtaaaagttgttgatgaattggtcaaagtaatggggcggcataagccagaaaatatcgttattgaaatggcacgtgaaaatcagacaactcaaaagggccagaaaaattcgcgagagcgtatgaaacgaatcgaagaaggtatcaaagaattaggaagtcagattcttaaagagcatcctgttgaaaatactcaattgcaaaatgaaaagctctatctctattatctccaaaatggaagagacatgtatgtggaccaagaattagatattaatcgtttaagtgattatgatgtcgatcacattgttccacaaagtttccttaaagacgattcaatagacaataaggtcttaacgcgttctgataaaaatcgtggtaaatcggataacgttccaagtgaagaagtagtcaaaaagatgaaaaactattggagacaacttctaaacgccaagttaatcactcaacgtaagtttgataatttaacgaaagctgaacgtggaggtttgagtgaacttgataaagctggttttatcaaacgccaattggttgaaactcgccaaatcactaagcatgtggcacaaattttggatagtcgcatgaatactaaatacgatgaaaatgataaacttattcgagaggttaaagtgattaccttaaaatctaaattagtttctgacttccgaaaagatttccaattctataaagtacgtgagattaacaattaccatcatgcccatgatgcgtatctaaatgccgtcgttggaactgctttgattaagaaatatccaaaacttgaatcggagtttgtctatggtgattataaagtttatgatgttcgtaaaatgattgctaagtctgagcaagaaataggcaaagcaaccgcaaaatatttcttttactctaatatcatgaacttcttcaaaacagaaattacacttgcaaatggagagattcgcaaacgccctctaatcgaaactaatggggaaactggagaaattgtctgggataaagggcgagattttgccacagtgcgcaaagtattgtccatgccccaagtcaatattgtcaagaaaacagaagtacagacaggcggattctccaaggagtcaattttaccaaaaagaaattcggacaagcttattgctcgtaaaaaagactgggatccaaaaaaatatggtggttttgatagtccaacggtagcttattcagtcctagtggttgctaaggtggaaaaagggaaatcgaagaagttaaaatccgttaaagagttactagggatcacaattatggaaagaagttcctttgaaaaaaatccgattgactttttagaagctaaaggatataaggaagttaaaaaagacttaatcattaaactacctaaatatagtctttttgagttagaaaacggtcgtaaacggatgctggctagtgccggagaattacaaaaaggaaatgagctggctctgccaagcaaatatgtgaattttttatatttagctagtcattatgaaaagttgaagggtagtccagaagataacgaacaaaaacaattgtttgtggagcagcataagcattatttagatgagattattgagcaaatcagtgaattttctaagcgtgttattttagcagatgccaatttagataaagttcttagtgcatataacaaacatagagacaaaccaatacgtgaacaagcagaaaatattattcatttatttacgttgacgaatcttggagctcccgctgcttttaaatattttgatacaacaattgatcgtaaacgatatacgtctacaaaagaagttttagatgccactcttatccatcaatccatcactggtctttatgaaacacgcattgatttgagtcagctaggaggtgactgaatggataagaaatactcaataggcttagatatcggcacaaatagcgtcggatgggcggtgatcactgatgaatataaggttccgtctaaaaagttcaaggttctgggaaatacagaccgccacagtatcaaaaaaaatcttataggggctcttttatttgacagtggagagacagcggaagcgactcgtctcaaacggacagctcgtagaaggtatacacgtcggaagaatcgtatttgttatctacaggagattttttcaaatgagatggcgaaagtagatgatagtttctttcatcgacttgaagagtcttttttggtggaagaagacaagaagcatgaacgtcatcctatttttggaaatatagtagatgaagttgcttatcatgagaaatatccaactatctatcatctgcgaaaaaaattggtagattctactgataaagcggatttgcgcttaatctatttggccttagcgcatatgattaagtttcgtggtcattttttgattgagggagatttaaatcctgataatagtgatgtggacaaactatttatccagttggtacaaacctacaatcaattatttgaagaaaaccctattaacgcaagtggagtagatgctaaagcgattctttctgcacgattgagtaaatcaagacgattagaaaatctcattgctcagctccccggtgagaagaaaaatggcttatttgggaatctcattgctttgtcattgggtttgacccctaattttaaatcaaattttgatttggcagaagatgctaaattacagctttcaaaagatacttacgatgatgatttagataatttattggcgcaaattggagatcaatatgctgatttgtttttggcagctaagaatttatcagatgctattttactttcagatatcctaagagtaaatactgaaataactaaggctcccctatcagcttcaatgattaaacgctacgatgaacatcatcaagacttgactcttttaaaagctttagttcgacaacaacttccagaaaagtataaagaaatcttttttgatcaatcaaaaaacggatatgcaggttatattgatgggggagctagccaagaagaattttataaatttatcaaaccaattttagaaaaaatggatggtactgaggaattattggtgaaactaaatcgtgaagatttgctgcgcaagcaacggacctttgacaacggctctattccccatcaaattcacttgggtgagctgcatgctattttgagaagacaagaagacttttatccatttttaaaagacaatcgtgagaagattgaaaaaatcttgacttttcgaattccttattatgttggtccattggcgcgtggcaatagtcgttttgcatggatgactcggaagtctgaagaaacaattaccccatggaattttgaagaagttgtcgataaaggtgcttcagctcaatcatttattgaacgcatgacaaactttgataaaaatcttccaaatgaaaaagtactaccaaaacatagtttgctttatgagtattttacggtttataacgaattgacaaaggtcaaatatgttactgaaggaatgcgaaaaccagcatttctttcaggtgaacagaagaaagccattgttgatttactcttcaaaacaaatcgaaaagtaaccgttaagcaattaaaagaagattatttcaaaaaaatagaatgttttgatagtgttgaaatttcaggagttgaagatagatttaatgcttcattaggtacctaccatgatttgctaaaaattattaaagataaagattttttggataatgaagaaaatgaagatatcttagaggatattgttttaacattgaccttatttgaagatagggagatgattgaggaaagacttaaaacatatgctcacctctttgatgataaggtgatgaaacagcttaaacgtcgccgttatactggttggggacgtttgtctcgaaaattgattaatggtattagggataagcaatctggcaaaacaatattagattttttgaaatcagatggttttgccaatcgcaattttatgcagctgatccatgatgatagtttgacatttaaagaagacattcaaaaagcacaagtgtctggacaaggcgatagtttacatgaacatattgcaaatttagctggtagccctgctattaaaaaaggtattttacagactgtaaaagttgttgatgaattggtcaaagtaatggggcggcataagccagaaaatatcgttattgaaatggcacgtgaaaatcagacaactcaaaagggccagaaaaattcgcgagagcgtatgaaacgaatcgaagaaggtatcaaagaattaggaagtcagattcttaaagagcatcctgttgaaaatactcaattgcaaaatgaaaagctctatctctattatctccaaaatggaagagacatgtatgtggaccaagaattagatattaatcgtttaagtgattatgatgtcgatcacattgttccacaaagtttccttaaagacgattcaatagacaataaggtcttaacgcgttctgataaaaatcgtggtaaatcggataacgttccaagtgaagaagtagtcaaaaagatgaaaaactattggagacaacttctaaacgccaagttaatcactcaacgtaagtttgataatttaacgaaagctgaacgtggaggtttgagtgaacttgataaagctggttttatcaaacgccaattggttgaaactcgccaaatcactaagcatgtggcacaaattttggatagtcgcatgaatactaaatacgatgaaaatgataaacttattcgagaggttaaagtgattaccttaaaatctaaattagtttctgacttccgaaaagatttccaattctataaagtacgtgagattaacaattaccatcatgcccatgatgcgtatctaaatgccgtcgttggaactgctttgattaagaaatatccaaaacttgaatcggagtttgtctatggtgattataaagtttatgatgttcgtaaaatgattgctaagtctgagcaagaaataggcaaagcaaccgcaaaatatttcttttactctaatatcatgaacttcttcaaaacagaaattacacttgcaaatggagagattcgcaaacgccctctaatcgaaactaatggggaaactggagaaattgtctgggataaagggcgagattttgccacagtgcgcaaagtattgtccatgccccaagtcaatattgtcaagaaaacagaagtacagacaggcggattctccaaggagtcaattttaccaaaaagaaattcggacaagcttattgctcgtaaaaaagactgggatccaaaaaaatatggtggttttgatagtccaacggtagcttattcagtcctagtggttgctaaggtggaaaaagggaaatcgaagaagttaaaatccgttaaagagttactagggatcacaattatggaaagaagttcctttgaaaaaaatccgattgactttttagaagctaaaggatataaggaagttaaaaaagacttaatcattaaactacctaaatatagtctttttgagttagaaaacggtcgtaaacggatgctggctagtgccggagaattacaaaaaggaaatgagctggctctgccaagcaaatatgtgaattttttatatttagctagtcattatgaaaagttgaagggtagtccagaagataacgaacaaaaacaattgtttgtggagcagcataagcattatttagatgagattattgagcaaatcagtgaattttctaagcgtgttattttagcagatgccaatttagataaagttcttagtgcatataacaaacatagagacaaaccaatacgtgaacaagcagaaaatattattcatttatttacgttgacgaatcttggagctcccgctgcttttaaatattttgatacaacaattgatcgtaaacgatatacgtctacaaaagaagttttagatgccactcttatccatcaatccatcactggtctttatgaaacacgcattgatttgagtcagctaggaggtgactgaatggataagaaatactcaataggcttagatatcggcacaaatagcgtcggatgggcggtgatcactgatgaatataaggttccgtctaaaaagttcaaggttctgggaaatacagaccgccacagtatcaaaaaaaatcttataggggctcttttatttgacagtggagagacagcggaagcgactcgtctcaaacggacagctcgtagaaggtatacacgtcggaagaatcgtatttgttatctacaggagattttttcaaatgagatggcgaaagtagatgatagtttctttcatcgacttgaagagtcttttttggtggaagaagacaagaagcatgaacgtcatcctatttttggaaatatagtagatgaagttgcttatcatgagaaatatccaactatctatcatctgcgaaaaaaattggtagattctactgataaagcggatttgcgcttaatctatttggccttagcgcatatgattaagtttcgtggtcattttttgattgagggagatttaaatcctgataatagtgatgtggacaaactatttatccagttggtacaaacctacaatcaattatttgaagaaaaccctattaacgcaagtggagtagatgctaaagcgattctttctgcacgattgagtaaatcaagacgattagaaaatctcattgctcagctccccggtgagaagaaaaatggcttatttgggaatctcattgctttgtcattgggtttgacccctaattttaaatcaaattttgatttggcagaagatgctaaattacagctttcaaaagatacttacgatgatgatttagataatttattggcgcaaattggagatcaatatgctgatttgtttttggcagctaagaatttatcagatgctattttactttcagatatcctaagagtaaatactgaaataactaaggctcccctatcagcttcaatgattaaacgctacgatgaacatcatcaagacttgactcttttaaaagctttagttcgacaacaacttccagaaaagtataaagaaatcttttttgatcaatcaaaaaacggatatgcaggttatattgatgggggagctagccaagaagaattttataaatttatcaaaccaattttagaaaaaatggatggtactgaggaattattggtgaaactaaatcgtgaagatttgctgcgcaagcaacggacctttgacaacggctctattccccatcaaattcacttgggtgagctgcatgctattttgagaagacaagaagacttttatccatttttaaaagacaatcgtgagaagattgaaaaaatcttgacttttcgaattccttattatgttggtccattggcgcgtggcaatagtcgttttgcatggatgactcggaagtctgaagaaacaattaccccatggaattttgaagaagttgtcgataaaggtgcttcagctcaatcatttattgaacgcatgacaaactttgataaaaatcttccaaatgaaaaagtactaccaaaacatagtttgctttatgagtattttacggtttataacgaattgacaaaggtcaaatatgttactgaaggaatgcgaaaaccagcatttctttcaggtgaacagaagaaagccattgttgatttactcttcaaaacaaatcgaaaagtaaccgttaagcaattaaaagaagattatttcaaaaaaatagaatgttttgatagtgttgaaatttcaggagttgaagatagatttaatgcttcattaggtacctaccatgatttgctaaaaattattaaagataaagattttttggataatgaagaaaatgaagatatcttagaggatattgttttaacattgaccttatttgaagatagggagatgattgaggaaagacttaaaacatatgctcacctctttgatgataaggtgatgaaacagcttaaacgtcgccgttatactggttggggacgtttgtctcgaaaattgattaatggtattagggataagcaatctggcaaaacaatattagattttttgaaatcagatggttttgccaatcgcaattttatgcagctgatccatgatgatagtttgacatttaaagaagacattcaaaaagcacaagtgtctggacaaggcgatagtttacatgaacatattgcaaatttagctggtagccctgctattaaaaaaggtattttacagactgtaaaagttgttgatgaattggtcaaagtaatggggcggcataagccagaaaatatcgttattgaaatggcacgtgaaaatcagacaactcaaaagggccagaaaaattcgcgagagcgtatgaaacgaatcgaagaaggtatcaaagaattaggaagtcagattcttaaagagcatcctgttgaaaatactcaattgcaaaatgaaaagctctatctctattatctccaaaatggaagagacatgtatgtggaccaagaattagatattaatcgtttaagtgattatgatgtcgatcacattgttccacaaagtttccttaaagacgattcaatagacaataaggtcttaacgcgttctgataaaaatcgtggtaaatcggataacgttccaagtgaagaagtagtcaaaaagatgaaaaactattggagacaacttctaaacgccaagttaatcactcaacgtaagtttgataatttaacgaaagctgaacgtggaggtttgagtgaacttgataaagctggttttatcaaacgccaattggttgaaactcgccaaatcactaagcatgtggcacaaattttggatagtcgcatgaatactaaatacgatgaaaatgataaacttattcgagaggttaaagtgattaccttaaaatctaaattagtttctgacttccgaaaagatttccaattctataaagtacgtgagattaacaattaccatcatgcccatgatgcgtatctaaatgccgtcgttggaactgctttgattaagaaatatccaaaacttgaatcggagtttgtctatggtgattataaagtttatgatgttcgtaaaatgattgctaagtctgagcaagaaataggcaaagcaaccgcaaaatatttcttttactctaatatcatgaacttcttcaaaacagaaattacacttgcaaatggagagattcgcaaacgccctctaatcgaaactaatggggaaactggagaaattgtctgggataaagggcgagattttgccacagtgcgcaaagtattgtccatgccccaagtcaatattgtcaagaaaacagaagtacagacaggcggattctccaaggagtcaattttaccaaaaagaaattcggacaagcttattgctcgtaaaaaagactgggatccaaaaaaatatggtggttttgatagtccaacggtagcttattcagtcctagtggttgctaaggtggaaaaagggaaatcgaagaagttaaaatccgttaaagagttactagggatcacaattatggaaagaagttcctttgaaaaaaatccgattgactttttagaagctaaaggatataaggaagttaaaaaagacttaatcattaaactacctaaatatagtctttttgagttagaaaacggtcgtaaacggatgctggctagtgccggagaattacaaaaaggaaatgagctggctctgccaagcaaatatgtgaattttttatatttagctagtcattatgaaaagttgaagggtagtccagaagataacgaacaaaaacaattgtttgtggagcagcataagcattatttagatgagattattgagcaaatcagtgaattttctaagcgtgttattttagcagatgccaatttagataaagttcttagtgcatataacaaacatagagacaaaccaatacgtgaacaagcagaaaatattattcatttatttacgttgacgaatcttggagctcccgctgcttttaaatattttgatacaac

SEQ ID NO: 92 - DNA, 4107 bp, Artificial Sequence
  codon optimized S. pyogenes Cas9
atggataaaaaatacagcattggtctggatatcggaaccaacagcgttgggtgggcagtaataacagatgaatacaaagtgccgtcaaaaaaatttaaggttctggggaatacagatcgccacagcataaaaaagaatctgattggggcattgctgtttgattcgggtgagacagctgaggccacgcgtctgaaacgtacagcaagaagacgttacacacgtcgtaaaaatcgtatttgctacttacaggaaattttttctaacgaaatggccaaggtagatgatagtttcttccatcgtctcgaagaatcttttctggttgaggaagataaaaaacacgaacgtcaccctatctttggcaatatcgtggatgaagtggcctatcatgaaaaataccctacgatttatcatcttcgcaagaagttggttgatagtacggacaaagcggatctgcgtttaatctatcttgcgttagcgcacatgatcaaatttcgtggtcatttcttaattgaaggtgatctgaatcctgataactctgatgtggacaaattgtttatacaattagtgcaaacctataatcagctgttcgaggaaaaccccattaatgcctctggagttgatgccaaagcgattttaagcgcgagactttctaagtcccggcgtctggagaatctgatcgcccagttaccaggggaaaagaaaaatggtctgtttggtaatctgattgccctcagtctggggcttaccccgaacttcaaatccaattttgacctggctgaggacgcaaagctgcagctgagcaaagatacttatgatgatgacctcgacaatctgctcgcccagattggtgaccaatatgcggatctgtttctggcagcgaagaatctttcggatgctatcttgctgtcggatattctgcgtgttaataccgaaatcaccaaagcgcctctgtctgcaagtatgatcaagagatacgacgagcaccaccaggacctgactcttcttaaggcactggtacgccaacagcttccggagaaatacaaagaaatattcttcgaccagtccaagaatggttacgcgggctacatcgatggtggtgcatcacaggaagagttctataaatttattaaaccaatccttgagaaaatggatggcacggaagagttacttgttaaacttaaccgcgaagacttgcttagaaagcaacgtacattcgacaacggctccatcccacaccagattcatttaggtgaacttcacgccatcttgcgcagacaagaagatttctatcccttcttaaaagacaatcgggagaaaatcgagaagatcctgacgttccgcattccctattatgtcggtcccctggcacgtggtaattctcggtttgcctggatgacgcgcaaaagtgaggaaaccatcaccccttggaactttgaagaagtcgtggataaaggtgctagcgcgcagtcttttatagaaagaatgacgaacttcgataaaaacttgcccaacgaaaaagtcctgcccaagcactctcttttatatgagtactttactgtgtacaacgaactgactaaagtgaaatacgttacggaaggtatgcgcaaacctgcctttcttagtggcgagcagaaaaaagcaattgtcgatcttctctttaaaacgaatcgcaaggtaactgtaaaacagctgaaggaagattatttcaaaaagatcgaatgctttgattctgtcgagatctcgggtgtcgaagatcgtttcaacgcttccttagggacctatcatgatttgctgaagataataaaagacaaagactttctcgacaatgaagaaaatgaagatattctggaggatattgttttgaccttgaccttattcgaagatagagagatgatcgaggagcgcttaaaaacctatgcccacctgtttgatgacaaagtcatgaagcaattaaagcgccgcagatatacggggtggggccgcttgagccgcaagttgattaacggtattagagacaagcagagcggaaaaactatcctggatttcctcaaatctgacggatttgcgaaccgcaattttatgcagcttatacatgatgattcgcttacattcaaagaggatattcagaaggctcaggtgtctgggcaaggtgattcactccacgaacatatagcaaatttggccggctctcctgcgattaagaaggggatcctgcaaacagttaaagttgtggatgaacttgtaaaagtaatgggccgccacaagccggagaatatcgtgatagaaatggcgcgcgagaatcaaacgacacaaaaaggtcaaaagaactcaagagagagaatgaagcgcattgaggaggggataaaggaacttggatctcaaattctgaaagaacatccagttgaaaacactcagctgcaaaatgaaaaattgtacctgtactacctgcagaatggaagagacatgtacgtggatcaggaattggatatcaatagactctcggactatgacgtagatcacattgtccctcagagcttcctcaaggatgattctatagataataaagtacttacgagatcggacaaaaatcgcggtaaatcggataacgtcccatcggaggaagtcgttaaaaagatgaaaaactattggcgtcaactgctgaacgccaagctgatcacacagcgtaagtttgataatctgactaaagccgaacgcggtggtcttagtgaactcgataaagcaggatttataaaacggcagttagtagaaacgcgccaaattacgaaacacgtggctcagatcctcgattctagaatgaatacaaagtacgatgaaaacgataaactgatccgtgaagtaaaagtcattaccttaaaatctaaacttgtgtccgatttccgcaaagattttcagttttacaaggtccgggaaatcaataactatcaccatgcacatgatgcatatttaaatgcggttgtaggcacggcccttattaagaaataccctaaactcgaaagtgagtttgtttatggggattataaagtgtatgacgttcgcaaaatgatcgcgaaatcagaacaggaaatcggtaaggctaccgctaaatactttttttattccaacattatgaatttttttaagaccgaaataactctcgcgaatggtgaaatccgtaaacggcctcttatagaaaccaatggtgaaacgggagaaatcgtttgggataaaggtcgtgactttgccaccgttcgtaaagtcctctcaatgccgcaagttaacattgtcaagaagacggaagttcaaacagggggattctccaaagaatctatcctgccgaagcgtaacagtgataaacttattgccagaaaaaaagattgggatccaaaaaaatacggaggctttgattcccctaccgtcgcgtatagtgtgctggtggttgctaaagtcgagaaagggaaaagcaagaaattgaaatcagttaaagaactgctgggtattacaattatggaaagatcgtcctttgagaaaaatccgatcgactttttagaggccaaggggtataaggaagtgaaaaaagatctcatcatcaaattaccgaagtatagtctttttgagctggaaaacggcagaaaaagaatgctggcctccgcgggcgagttacagaagggaaatgagctggcgctgccttccaaatatgttaattttctgtaccttgccagtcattatgagaaactgaagggcagccccgaagataacgaacagaaacaattattcgtggaacagcataagcactatttagatgaaattatagagcaaattagtgaattttctaagcgcgttatcctcgcggatgctaatttagacaaagtactgtcagcttataataaacatcgggataagccgattagagaacaggccgaaaatatcattcatttgtttaccttaaccaaccttggagcaccagctgccttcaaatatttcgataccacaattgatcgtaaacggtatacaagtacaaaagaagtcttggacgcaaccctcattcatcaatctattactggattatatgagacacgcattgatctttcacagctgggcggagactaa

SEQ ID NO: 93 - DNA, 607 bp, Bacillus subtilis
attcctccattttcttctgctatcaaaataacagactcgtgattttccaaacgagctttcaaaaaagcctctgccccttgcaaatcggatgcctgtctataaaattcccgatattggttaaacagcggcgcaatggcggccgcatctgatgtctttgcttggcgaatgttcatcttatttcttcctccctctcaataattttttcattctatcccttttctgtaaagtttatttttcagaatacttttatcatcatgctttgaaaaaatatcacgataatatccattgttctcacggaagcacacgcaggtcatttgaacgaattttttcgacaggaatttgccgggactcaggagcatttaacctaaaaaagcatgacatttcagcataatgaacatttactcatgtctattttcgttcttttctgtatgaaaatagttatttcgagtctctacggaaatagcgagagatgatatacctaaatagagataaaatcatctcaaaaaaatgggtctactaaaatattattccatctattacaataaattcacagaatagtcttttaagtaagtctactctgaatttttttaaaaggagagggtaacta

SEQ ID NO: 94 - DNA, 138 bp, Bacillus subtilis
tattgaaaatactgacgaggttatataagatgaaaataagttagtttgtttaaacaacaaactaataggtgatgtacttactatatgaaataaaatgcatctgtatttgaatgaatttatttttaagggggaaatcac

SEQ ID NO: 95 - DNA, 177 bp, Artificial Sequence
  spac promoter
ggtagcccttgcctacctagcttccaagaaagatatcctaacagcacaagagcggaaagatgttttgttctacatccagaacaacctctgctaaaattcctgaaaaattttgcaaaaagttgttgactttatctacaaggtgtggcataatgtgtggaattgtgagcgctcacaatt

SEQ ID NO: 96 - DNA, 100 bp, Artificial Sequence
  hyper-spank promoter
ctcgagggtaaatgtgagcactcacaattcattttgcaaaagttgttgactttatctacaaggtgtggcataatgtgtgtaattgtgagcggataacaat

SEQ ID NO: 97 - DNA, 237 bp, Bacillus subtilis
ggagttctgagaattggtatgccttataagtccaattaacagttgaaaacctgcataggagagctatgcgggttttttattttacataatgatacataatttaccgaaacttgcggaacataattgaggaatcatagaattttgtcaaaataattttattgacaacgtcttattaacgttgatataatttaaattttatttgacaaaaatgggctcgtgttgtacaataaatgtagt

SEQ ID NO: 98 - DNA, 270 bp, Bacillus subtilis
gaattcgagctcggtaccgatcttaacatttttcccctatcatttttccgtcttcatttgtcattttttccagaaaaaatcgcgtcattcgactcatgtctaatccaacacgtgtctctcggcttatcccctgacaccgcccgccgacagcccgcatgggacgattctatcaattcagccgcggagtctagttttatattgcagaatgcgagattgctggtttattataacaatataagttttcattattttcaaaaagggggatttatt

SEQ ID NO: 99 - DNA, 56 bp, T5 phage
aagaatcataaaaaatttatttgctttcaggaaaatttttctgtataatagattca

SEQ ID NO: 100 - DNA, 173 bp, Bacillus subtilis
gctattgtaacataatcggtacgggggtgaaaaagctaacggaaaagggagcggaaaagaatgatgtaagcgtgaaaaattttttatcttatcacttgaaattggaagggagattctttattataagaattgtggaattgtgagcggataacaattcccaattaaaggaggaa

SEQ ID NO: 101 - DNA, 231 bp, Bacillus subtilis
aagcttctcatcaatgatttgaattggagctcgggctggccgtcctattgaattaaaaagccgggctctgcccccggctttttttaaaagaaaagattgacagtataatagtcaattactataataaaattgttcgtacaaatatttatttataggtttattttctatcattagtacgtatcttttgtatttgaaagcgttttattttatgagaaaggggcagtttacatg

SEQ ID NO: 102 - DNA, 231 bp, Bacillus licheniformis
ttctgaaatctgtcaaaaaaaataaaaaacataccggaaattaaattgacagtttttttcataatgatataatgaagttgttcgtacaaatatgtttttgatgttagttgtacgtacatataatcgcgatacagtttgagatcaaggtatgatttatgtttttttgtaagcgttttaatagtttgctattctacacagacaccataaagacgaggaggaggaagctatttg

SEQ ID NO: 103 - DNA, 95 bp, lambda phage
gactcctgttgatagatccagtaatgacctcagaactccatctggatttgttcagaacgctcggttgccgccgggcgttttttattggtgagaat

SEQ ID NO: 104 - DNA, 4809 bp, Artificial Sequence
  cas9 expression cassette
attcctccattttcttctgctatcaaaataacagactcgtgattttccaaacgagctttcaaaaaagcctctgccccttgcaaatcggatgcctgtctataaaattcccgatattggttaaacagcggcgcaatggcggccgcatctgatgtctttgcttggcgaatgttcatcttatttcttcctccctctcaataattttttcattctatcccttttctgtaaagtttatttttcagaatacttttatcatcatgctttgaaaaaatatcacgataatatccattgttctcacggaagcacacgcaggtcatttgaacgaattttttcgacaggaatttgccgggactcaggagcatttaacctaaaaaagcatgacatttcagcataatgaacatttactcatgtctattttcgttcttttctgtatgaaaatagttatttcgagtctctacggaaatagcgagagatgatatacctaaatagagataaaatcatctcaaaaaaatgggtctactaaaatattattccatctattacaataaattcacagaatagtcttttaagtaagtctactctgaatttttttaaaaggagagggtaactaatggataaaaaatacagcattggtctggatatcggaaccaacagcgttgggtgggcagtaataacagatgaatacaaagtgccgtcaaaaaaatttaaggttctggggaatacagatcgccacagcataaaaaagaatctgattggggcattgctgtttgattcgggtgagacagctgaggccacgcgtctgaaacgtacagcaagaagacgttacacacgtcgtaaaaatcgtatttgctacttacaggaaattttttctaacgaaatggccaaggtagatgatagtttcttccatcgtctcgaagaatcttttctggttgaggaagataaaaaacacgaacgtcaccctatctttggcaatatcgtggatgaagtggcctatcatgaaaaataccctacgatttatcatcttcgcaagaagttggttgatagtacggacaaagcggatctgcgtttaatctatcttgcgttagcgcacatgatcaaatttcgtggtcatttcttaattgaaggtgatctgaatcctgataactctgatgtggacaaattgtttatacaattagtgcaaacctataatcagctgttcgaggaaaaccccattaatgcctctggagttgatgccaaagcgattttaagcgcgagactttctaagtcccggcgtctggagaatctgatcgcccagttaccaggggaaaagaaaaatggtctgtttggtaatctgattgccctcagtctggggcttaccccgaacttcaaatccaattttgacctggctgaggacgcaaagctgcagctgagcaaagatacttatgatgatgacctcgacaatctgctcgcccagattggtgaccaatatgcggatctgtttctggcagcgaagaatctttcggatgctatcttgctgtcggatattctgcgtgttaataccgaaatcaccaaagcgcctctgtctgcaagtatgatcaagagatacgacgagcaccaccaggacctgactcttcttaaggcactggtacgccaacagcttccggagaaatacaaagaaatattcttcgaccagtccaagaatggttacgcgggctacatcgatggtggtgcatcacaggaagagttctataaatttattaaaccaatccttgagaaaatggatggcacggaagagttacttgttaaacttaaccgcgaagacttgcttagaaagcaacgtacattcgacaacggctccatcccacaccagattcatttaggtgaacttcacgccatcttgcgcagacaagaagatttctatcccttcttaaaagacaatcgggagaaaatcgagaagatcctgacgttccgcattccctattatgtcggtcccctggcacgtggtaattctcggtttgcctggatgacgcgcaaaagtgaggaaaccatcaccccttggaactttgaagaagtcgtggataaaggtgctagcgcgcagtcttttatagaaagaatgacgaacttcgataaaaacttgcccaacgaaaaagtcctgcccaagcactctcttttatatgagtactttactgtgtacaacgaactgactaaagtgaaatacgttacggaaggtatgcgcaaacctgcctttcttagtggcgagcagaaaaaagcaattgtcgatcttctctttaaaacgaatcgcaaggtaactgtaaaacagctgaaggaagattatttcaaaaagatcgaatgctttgattctgtcgagatctcgggtgtcgaagatcgtttcaacgcttccttagggacctatcatgatttgctgaagataataaaagacaaagactttctcgacaatgaagaaaatgaagatattctggaggatattgttttgaccttgaccttattcgaagatagagagatgatcgaggagcgcttaaaaacctatgcccacctgtttgatgacaaagtcatgaagcaattaaagcgccgcagatatacggggtggggccgcttgagccgcaagttgattaacggtattagagacaagcagagcggaaaaactatcctggatttcctcaaatctgacggatttgcgaaccgcaattttatgcagcttatacatgatgattcgcttacattcaaagaggatattcagaaggctcaggtgtctgggcaaggtgattcactccacgaacatatagcaaatttggccggctctcctgcgattaagaaggggatcctgcaaacagttaaagttgtggatgaacttgtaaaagtaatgggccgccacaagccggagaatatcgtgatagaaatggcgcgcgagaatcaaacgacacaaaaaggtcaaaagaactcaagagagagaatgaagcgcattgaggaggggataaaggaacttggatctcaaattctgaaagaacatccagttgaaaacactcagctgcaaaatgaaaaattgtacctgtactacctgcagaatggaagagacatgtacgtggatcaggaattggatatcaatagactctcggactatgacgtagatcacattgtccctcagagcttcctcaaggatgattctatagataataaagtacttacgagatcggacaaaaatcgcggtaaatcggataacgtcccatcggaggaagtcgttaaaaagatgaaaaactattggcgtcaactgctgaacgccaagctgatcacacagcgtaagtttgataatctgactaaagccgaacgcggtggtcttagtgaactcgataaagcaggatttataaaacggcagttagtagaaacgcgccaaattacgaaacacgtggctcagatcctcgattctagaatgaatacaaagtacgatgaaaacgataaactgatccgtgaagtaaaagtcattaccttaaaatctaaacttgtgtccgatttccgcaaagattttcagttttacaaggtccgggaaatcaataactatcaccatgcacatgatgcatatttaaatgcggttgtaggcacggcccttattaagaaataccctaaactcgaaagtgagtttgtttatggggattataaagtgtatgacgttcgcaaaatgatcgcgaaatcagaacaggaaatcggtaaggctaccgctaaatactttttttattccaacattatgaatttttttaagaccgaaataactctcgcgaatggtgaaatccgtaaacggcctcttatagaaaccaatggtgaaacgggagaaatcgtttgggataaaggtcgtgactttgccaccgttcgtaaagtcctctcaatgccgcaagttaacattgtcaagaagacggaagttcaaacagggggattctccaaagaatctatcctgccgaagcgtaacagtgataaacttattgccagaaaaaaagattgggatccaaaaaaatacggaggctttgattcccctaccgtcgcgtatagtgtgctggtggttgctaaagtcgagaaagggaaaagcaagaaattgaaatcagttaaagaactgctgggtattacaattatggaaagatcgtcctttgagaaaaatccgatcgactttttagaggccaaggggtataaggaagtgaaaaaagatctcatcatcaaattaccgaagtatagtctttttgagctggaaaacggcagaaaaagaatgctggcctccgcgggcgagttacagaagggaaatgagctggcgctgccttccaaatatgttaattttctgtaccttgccagtcattatgagaaactgaagggcagccccgaagataacgaacagaaacaattattcgtggaacagcataagcactatttagatgaaattatagagcaaattagtgaattttctaagcgcgttatcctcgcggatgctaatttagacaaagtactgtcagcttataataaacatcgggataagccgattagagaacaggccgaaaatatcattcatttgtttaccttaaccaaccttggagcaccagctgccttcaaatatttcgataccacaattgatcgtaaacggtatacaagtacaaaagaagtcttggacgcaaccctcattcatcaatctattactggattatatgagacacgcattgatctttcacagctgggcggagactaagactcctgttgatagatccagtaatgacctcagaactccatctggatttgttcagaacgctcggttgccgccgggcgttttttattggtgagaat

SEQ ID NO: 105 - DNA, 23 bp, Bacillus licheniformis
aatggctgcggctctggaaatgg

SEQ ID NO: 106 - DNA, 17 bp, Artificial Sequence
  17 bp VT
ggctgcggctctggaaa

SEQ ID NO: 107 - DNA, 18 bp, Artificial Sequence
  18bp VT
tggctgcggctctggaaa

SEQ ID NO: 108 - DNA, 19 bp, Artificial Sequence
  19bp VT
atggctgcggctctggaaa

SEQ ID NO: 109 - DNA, 20 bp, Artificial Sequence
  20bp VT
aatggctgcggctctggaaa

SEQ ID NO: 110 - DNA, 76 bp, Artificial Sequence
  Cas9 endoncuclease recognition domain
gttttagagctagaaatagcaagttaaaataaggctagtccgttatcaacttgaaaaagtggcaccgagtcggtgc

SEQ ID NO: 111 - DNA, 96 bp, Artificial Sequence
  DNA encoding gRNA targeting duplication
aatggctgcggctctggaaagttttagagctagaaatagcaagttaaaataaggctagtccgttatcaacttgaaaaagtggcaccgagtcggtgc

SEQ ID NO: 112 - DNA, 368 bp, Artificial Sequence
  duplication gRNA expression cassette
ggtagcccttgcctacctagcttccaagaaagatatcctaacagcacaagagcggaaagatgttttgttctacatccagaacaacctctgctaaaattcctgaaaaattttgcaaaaagttgttgactttatctacaaggtgtggcataatgtgtggaattgtgagcgctcacaattaatggctgcggctctggaaagttttagagctagaaatagcaagttaaaataaggctagtccgttatcaacttgaaaaagtggcaccgagtcggtgcgactcctgttgatagatccagtaatgacctcagaactccatctggatttgttcagaacgctcggttgccgccgggcgttttttattggtgagaat

SEQ ID NO: 113 - DNA, 500 bp, Bacillus licheniformis
gtatgaggaactgatggcatctgcaggctatatcagcgcgtctacagtccaggaagcaagaagcagctatgattccatttacgacatcgtgtcacagtacgatttagaggacctttctctgtttgacagcgaaaagtggaaggtgctttcaaaaaaagacatcgaaaacctggacaaatatttcgactttctcgtgcaggaagcaagcagccgaaacaaaaactgaatacttctccgcggcacactctcctctctatcattttcgtctgtttacgatcctgctgttattttatcccttatgttaacttttgtcaatatttttcctgtctaagtatttcctatagtcaacatttgtattaaaatgttcatatcatgaatttgcgggggggatggcgatgacaaggttcggcgagcggctcaaagagctgagggaacaaagaagcctgtcggttaatcagcttgccatgtatgccggtgtgagcgccgcagccatttccaga

SEQ ID NO: 114 - DNA, 500 bp, Bacillus licheniformis
atcgaaaacggccaccgcggcgttcccaagcccgcgacgatcagaaaattggccgaggctctgaaaatgccgtacgagcagctcatggatattgccggttatatgagagctgacgagattcgcgaacagccgcgcggctatgtcacgatgcaggagatcgcggccaagcacggcgtcgaagacctgtggctgtttaaacccgagaaatgggactgtttgtcccgcgaagacctgctcaacctcgaacagtattttcattttttggttaatgaagcgaagaagcgccaatcataaaaagccgaatttcccttttaggagaagttcggcttttttcggctgccttaagcggcatccggattcggcgtcttgcctttatgatgcttaacggggctcagcgcacgctcgagccatcccatgaacagatcggcgatgatcgccatcagcgccgtcgggatcgcgcctgctagaatgatcgctgttccgttggtcgcgtttgatcc

SEQ ID NO: 115 - DNA, 1000 bp, Artificial Sequence
  rghR2 duplication editing template
gtatgaggaactgatggcatctgcaggctatatcagcgcgtctacagtccaggaagcaagaagcagctatgattccatttacgacatcgtgtcacagtacgatttagaggacctttctctgtttgacagcgaaaagtggaaggtgctttcaaaaaaagacatcgaaaacctggacaaatatttcgactttctcgtgcaggaagcaagcagccgaaacaaaaactgaatacttctccgcggcacactctcctctctatcattttcgtctgtttacgatcctgctgttattttatcccttatgttaacttttgtcaatatttttcctgtctaagtatttcctatagtcaacatttgtattaaaatgttcatatcatgaatttgcgggggggatggcgatgacaaggttcggcgagcggctcaaagagctgagggaacaaagaagcctgtcggttaatcagcttgccatgtatgccggtgtgagcgccgcagccatttccagaatcgaaaacggccaccgcggcgttcccaagcccgcgacgatcagaaaattggccgaggctctgaaaatgccgtacgagcagctcatggatattgccggttatatgagagctgacgagattcgcgaacagccgcgcggctatgtcacgatgcaggagatcgcggccaagcacggcgtcgaagacctgtggctgtttaaacccgagaaatgggactgtttgtcccgcgaagacctgctcaacctcgaacagtattttcattttttggttaatgaagcgaagaagcgccaatcataaaaagccgaatttcccttttaggagaagttcggcttttttcggctgccttaagcggcatccggattcggcgtcttgcctttatgatgcttaacggggctcagcgcacgctcgagccatcccatgaacagatcggcgatgatcgccatcagcgccgtcgggatcgcgcctgctagaatgatcgctgttccgttggtcgcgtttgatcc

SEQ ID NO: 116 - DNA, 20 bp, Bacillus licheniformis
gcgaatcgaaaacggaaagc

SEQ ID NO: 117 - DNA, 20 bp, Artificial Sequence
  rghR2 locus forward
gcgaatcgaaaacggaaagc

SEQ ID NO: 118 - DNA, 20 bp, Artificial Sequence
  rghR2 locus reverse
tcatcgcgatcggcattacg

SEQ ID NO: 119 - DNA, 1146 bp, Artificial Sequence
  Edited rghR2 locus
gcgaatcgaaaacggaaagcgcggcgtgccgaagccggcgacgatcagaaaactggcggacgctttgaaagtcccgtatgaggaactgatggcatctgcaggctatatcagcgcgtctacagtccaggaagcaagaagcagctatgattccatttacgacatcgtgtcacagtacgatttagaggacctttctctgtttgacagcgaaaagtggaaggtgctttcaaaaaaagacatcgaaaacctggacaaatatttcgactttctcgtgcaggaagcaagcagccgaaacaaaaactgaatacttctccgcggcacactctcctctctatcattttcgtctgtttacgatcctgctgttattttatcccttatgttaacttttgtcaatatttttcctgtctaagtatttcctatagtcaacatttgtattaaaatgttcatatcatgaatttgcgggggggatggcgatgacaaggttcggcgagcggctcaaagagctgagggaacaaagaagcctgtcggttaatcagcttgccatgtatgccggtgtgagcgccgcagccatttccagaatcgaaaacggccaccgcggcgttcccaagcccgcgacgatcagaaaattggccgaggctctgaaaatgccgtacgagcagctcatggatattgccggttatatgagagctgacgagattcgcgaacagccgcgcggctatgtcacgatgcaggagatcgcggccaagcacggcgtcgaagacctgtggctgtttaaacccgagaaatgggactgtttgtcccgcgaagacctgctcaacctcgaacagtattttcattttttggttaatgaagcgaagaagcgccaatcataaaaagccgaatttcccttttaggagaagttcggcttttttcggctgccttaagcggcatccggattcggcgtcttgcctttatgatgcttaacggggctcagcgcacgctcgagccatcccatgaacagatcggcgatgatcgccatcagcgccgtcgggatcgcgcctgctagaatgatcgctgttccgttggtcgcgtttgatcccctgacaatgatatccccgaggccgcctgcgccgacaaacgtgccgatggccgtaatgccgatcgcgatga

SEQ ID NO: 120 - DNA, 20 bp, Artificial Sequence
  rghR2 sequencing primer
tttcgactttctcgtgcagg

SEQ ID NO: 121 - DNA, 23 bp, Bacillus licheniformis
ctttccgatcacaagttgtccgg

SEQ ID NO: 122 - DNA, 23 bp, Bacillus licheniformis
tttccgatcacaagttgtccggg

SEQ ID NO: 123 - DNA, 23 bp, Bacillus licheniformis
aggcccggacaacttgtgatcgg

SEQ ID NO: 124 - DNA, 23 bp, Bacillus licheniformis
gagttttaaatggcgaaaggagg

SEQ ID NO: 125 - DNA, 23 bp, Bacillus licheniformis
ttaaatggcgaaaggaggcccgg

SEQ ID NO: 126 - DNA, 23 bp, Bacillus licheniformis
gcagagttttaaatggcgaaagg

SEQ ID NO: 127 - DNA, 23 bp, Bacillus licheniformis
acactcagcagagttttaaatgg

SEQ ID NO: 128 - DNA, 23 bp, Bacillus licheniformis
aactctgctgagtgtcgccgggg

SEQ ID NO: 129 - DNA, 23 bp, Bacillus licheniformis
aaaactctgctgagtgtcgccgg

SEQ ID NO: 130 - DNA, 23 bp, Bacillus licheniformis
aaactctgctgagtgtcgccggg

SEQ ID NO: 131 - DNA, 23 bp, Bacillus licheniformis
cattgaaatcggcgtatccccgg

SEQ ID NO: 132 - DNA, 23 bp, Bacillus licheniformis
cggggatacgccgatttcaatgg

SEQ ID NO: 133 - DNA, 23 bp, Bacillus licheniformis
aatcagcttgccattgaaatcgg

SEQ ID NO: 134 - DNA, 23 bp, Bacillus licheniformis
ttcaatggcaagctgatttaagg

SEQ ID NO: 135 - DNA, 23 bp, Bacillus licheniformis
gattgtgttcaatcatgtactgg

SEQ ID NO: 136 - DNA, 23 bp, Bacillus licheniformis
attagaaaggggagtaatcatgg

SEQ ID NO: 137 - DNA, 23 bp, Bacillus licheniformis
aaacataagagattagaaagggg

SEQ ID NO: 138 - DNA, 23 bp, Bacillus licheniformis
gaaacataagagattagaaaggg

SEQ ID NO: 139 - DNA, 23 bp, Bacillus licheniformis
agaaacataagagattagaaagg

SEQ ID NO: 140 - DNA, 1748 bp, Artificial Sequence
  amylase expression cassette
tcgctgataaacagctgacatcaactaaaagcttcattaaatactttgaaaaaagttgttgacttaaaagaagctaaatgttatagtaataaaacagaatagtcttttaagtaagtctactctgaatttttttaaaaggagagggtaaagaatgaaacaacaaaaacggctttacgcccgattgctgacgctgttatttgcgctcatcttcttgctgcctcattctgcagctagcgcagcagcgacaaacggaacaatgatgcagtatttcgagtggtatgtacctaacgacggccagcaatggaacagactgagaacagatgccccttacttgtcatctgttggtattaacgcagtatggacaccgccggcttataagggcacgtctcaagcagatgtggggtacggcccgtacgatctgtatgatttaggcgagtttaatcaaaaaggtacagtcagaacgaagtatggcacaaaaggagaacttaaatctgctgtcaacacgctgcattcaaatggaatccaagtgtatggtgatgtcgtgatgaatcataaagcaggtgctgattatacagaaaacgtaacggcggtggaggtgaatccgtctaatagatatcaggaaatcagcggcgaatataatattcaggcatggacaggcttcaactttccgggcagaggaacaacgtattctaactggaaatggcagtggttccattttgatggaacggattgggaccagagcagaagcctctctagaatcttcaaattcgatggaaaggcgtgggactggccggtttcttcagaaaacggaaattatgactatctgatgtacgcggactatgattatgaccatccggatgtcgtgaatgaaatgaaaaagtggggcgtctggtatgccaacgaagttgggttagatggatacagacttgacgcggtcaaacatattaaatttagctttctcaaagactgggtggataacgcaagagcagcgacgggaaaagaaatgtttacggttggcgaatattggcaaaatgatttaggggccctgaataactacctggcaaaggtaaattacaaccaatctctttttgatgcgccgttgcattacaacttttacgctgcctcaacagggggtggatattacgatatgagaaatattcttaataacacgttagtcgcaagcaatccgacaaaggctgttacgttagttgagaatcatgacacacagcctggacaatcactggaatcaacagtccaaccgtggtttaaaccgttagcctacgcgtttattctcacgagaagcggaggctatccttctgtattttatggagatatgtacggtacaaaaggaacgacaacaagagagatccctgctcttaaatctaaaatcgaacctttgcttaaggctagaaaagactatgcttatggaacacagagagactatattgataacccggatgtcattggctggacgagagaaggggactcaacgaaagccaagagcggtctggccacagtgattacagatgggccgggcggttcaaaaagaatgtatgttggcacgagcaatgcgggtgaaatctggtatgatttgacagggaatagaacagataaaatcacgattggaagcgatggctatgcaacatttcctgtcaataaggaatcagtttcagtatgggtgcagcaatgaaagcttctcgaggttaacagaggacggatttcctgaaggaaatccgtttttttatttt

SEQ ID NO: 141 - DNA, 1759 bp, Artificial Sequence
  amylase expression cassette
gtcgctgataaacagctgacatcaatatcctattttttcaaaaaatattttaaaaagttgttgacttaaaagaagctaaatgttatagtaataaaacagaatagtcttttaagtaagtctactctgaatttttttaaaaggagagggtaaagaatgaaacaacaaaaacggctttacgcccgattgctgacgctgttatttgcgctcatcttcttgctgcctcattctgcagctagcgcagccgcaccgtttaacggtaccatgatgcagtattttgaatggtacttgccggatgatggcacgttatggaccaaagtggccaatgaagccaacaacttatccagccttggcatcaccgctctttggctgccgcccgcttacaaaggaacaagccgcagcgacgtagggtacggagtatacgacttgtatgacctcggcgaattcaatcaaaaagggaccgtccgcacaaaatatggaacaaaagctcaatatcttcaagccattcaagccgcccacgccgctggaatgcaagtgtacgccgatgtcgtgttcgaccataaaggcggcgctgacggcacggaatgggtggacgccgtcgaagtcaatccgtccgaccgcaaccaagaaatctcgggcacctatcaaatccaagcatggacgaaatttgattttcccgggcggggcaacacctactccagctttaagtggcgctggtaccattttgacggcgttgattgggacgaaagccgaaaattaagccgcatttacaaattcaggggcatcggcaaagcgtgggattggccggtagacacagaaaacggaaactatgactacttaatgtatgccgaccttgatatggatcatcccgaagtcgtgaccgagctgaaaaactgggggaaatggtatgtcaacacaacgaacattgatgggttccggcttgatgccgtcaagcatattaagttcagtttttttcctgattggttgtcgtatgtgcgttctcagactggcaagccgctatttaccgtcggggaatattggagctatgacatcaacaagttgcacaattacattacgaaaacaaacggaacgatgtctttgtttgatgccccgttacacaacaaattttataccgcttccaaatcagggggcgcatttgatatgcgcacgttaatgaccaatactctcatgaaagatcaaccgacattggccgtcaccttcgttgataatcatgacaccgaacccggccaagcgcttcagtcatgggtcgacccatggttcaaaccgttggcttacgcctttattctaactcggcaggaaggatacccgtgcgtcttttatggtgactattatggcattccacaatataacattccttcgctgaaaagcaaaatcgatccgctcctcatcgcgcgcagggattatgcttacggaacgcaacatgattatcttgatcactccgacatcatcgggtggacaagggaaggggtcactgaaaaaccaggatccgggctggccgcactgatcaccgatgggccgggaggaagcaaatggatgtacgttggcaaacaacacgctggaaaagtgttctatgaccttaccggcaaccggagtgacaccgtcaccatcaacagtgatggatggggggaattcaaagtcaatggcggttcggtttcggtttgggttcctagaaaaacgacctaaaagcttctcgaggttaacagaggacggatttcctgaaggaaatccgtttttttatttt

SEQ ID NO: 142 - DNA, 1581 bp, Artificial Sequence
  expression cassette, synthetic sequence
gtcgctgataaacagctgacatcaatatcctattttttcaaaaaatattttaaaaagttgttgacttaaaagaagctaaatgttatagtaataaaacagaatagtcttttaagtaagtctactctgaatttttttaaaaggagagggtaaagaatgaaacaacaaaaacggctttacgcccgattgctgacgctgttatttgcgctcatcttcttgctgcctcattctgcagcttcagcagctgatcaagcaggaaaaagcccggcaggcgtcagatatcatggcggtgatgaaatcatccttcagggctttcattggaacgtcgtcagagaagcgccgtataactggtataacatcctgagacaacaagcgagcacaattgccgctgatggcttttccgcaatctggatgccggttccgtggagagattttagcagctggacggatggagataaaagcggaggcggcgaaggatatttttggcatgactttaacaaaaacggccgctatggaagcgatgctcaactgagacaagcagcaggagcacttggaggagcaggagtcaaagtcctgtacgatgtcgtcccgaaccatatgaaccgcttttatccggacaaagaaatcaatctgccggcaggccaaagattttggagaaacgattgcccggacccgggaaatggaccgaatgattgcgatgatggcgatagatttctgggcggcgaagcggatctgaatacaggccatccgcaaatctatggcatgtttcgggacgaatttacgaatctgagaagcggatatggagcgggcggatttcgctttgattttgtcagaggctatgccccggaaagagttgatagctggatgagcgattcagcggatagcagcttttgcgtcggcgaactttggaaagaaccgagcgaatatccgccgtgggattggagaaatacagcgagctggcagcagatcatcaaagattggagcgatagagcaaaatgcccggtctttgactttgccctgaaagaacgcatgcaaaatggaagcgtcgccgattggaaacatggcctgaacggaaatccggacccgagatggagagaagtcgccgtcacgtttgtcgataaccatgacacaggatatagcccgggacaaaatggaggacaacataaatggccgcttcaagatggccttatcagacaggcgtatgcctatatccttacatcaccgggaacaccggttgtttattggccgcatatgtatgattggggctatggcgatttcatccgccaactgatccaggttagaagaacagcaggagtcagagcggatagcgccattagctttcatagcggctatagcggacttgtcgctacagttagcggcagccaacaaacactggtcgtcgccctgaatagcgatctggcaaatccgggacaagttgctagcggcagctttagcgaagcagtcaatgccagcaatggccaagtcagagtctggagaagcggaagcggagatggaggaggaaatgacggcggctaaaagagcagagaggacggatttcctgaaggaaatccgtttttttatttt

SEQ ID NO: 143 - DNA, 1452 bp, Artificial Sequence
  Synthetic Cytophaga sp. variant #2 amylase expression cassette
gcagcgacaaacggaacaatgatgcagtatttcgagtggtatgtacctaacgacggccagcaatggaacagactgagaacagatgccccttacttgtcatctgttggtattacagcagtatggacaccgccggcttataagggcacgtctcaagcagatgtggggtacggcccgtacgatctgtatgatttaggcgagtttaatcaaaaaggtacagtcagaacgaagtatggcacaaaaggagaacttaaatctgctgtcaacacgctgcattcaaatggaatccaagtgtatggtgatgtcgtgatgaatcataaagcaggtgctgattatacagaaaacgtaacggcggtggaggtgaatccgtctaatagatatcaggaaacgagcggcgaatataatattcaggcatggacaggcttcaactttccgggcagaggaacaacgtattctaactggaaatggcagtggttccattttgatggaacggattgggaccagagcagaagcctctctagaatcttcaaattccatggaaaggcgtgggactggccggtttcttcagaaaacggaaattatgactatctgatgtacgcggactatgattatgaccatccggatgtcgtgaatgaaatgaaaaagtggggcgtctggtatgccaacgaagttgggttagatggatacagacttgacgcggtcaaacatattaaatttagctttctcaaagactgggtggataacgcaagagcagcgacgggaaaagaaatgtttacggttggcgaatattggcaaaatgatttaggggccctgaataactacctggcaaaggtaaattacaaccaatctctttttgatgcgccgttgcattacaacttttacgctgcctcaacagggggtggagcgtacgatatgagaaatattcttaataacacgttagtcgcaagcaatccgacaaaggctgttacgttagttgagaatcatgacacacagcctggacaatcactggaatcaacagtccaaccgtggtttaaaccgttagcctacgcgtttattctcacgagaagcggaggctatcctgcggtattttatggagatatgtacggtacaaaaggaacgacaacatatgagatccctgctcttaaatctaaaatcgaacctttgcttaaggctagaaaagactatgcttatggaacacagagagactatattgataacccggatgtcattggctggacgagagaaggggactcaacgaaagccaagagcggtctggccacagtgattacagatgggccgggcggttcaaaaagaatgtatgttggcacgagcaatgcgggtgaaatctggtatgatttgacagggaatagaacagataaaatcacgattggaagcgatggctatgcaacatttcctgtcaatgggggctcagtttcagtatgggtgcagcaatga

SEQ ID NO: 144 - DNA, 846 bp, Artificial Sequence
  synthetic allele glcT1 sequence
gtgaacagatcctttaccgttgaaaaggtactcaacaacaacgttttaatcgctctccatgatgattacagagaagttgtcttgattggcaaaggaatcggttttggtaaaaagcgcggagatcttatcgaacatgagaactacgaaaaaatgtttatcctggaaaatgataaggaacaatcgcagtataagaagctcttcacttatgtcgatgaaaaaatggttgatatcgccaatgatgtcatctaccatatcgcgcaaaaaatcggccagccgctgaacgaacacattcatgtcgccctgacggaccatatcgcatttgcagttaagcgtctagaaaagggatttgatatgaaaaatccgtttttgcttgagacggaatcgctttatccgaaggaatacgaagtcgccaaggaagccgtcgatatgattaatgaaaaatccgacattcagctgcctgaaggtgaaatcgggttcatcgcgcttcatatccacagtgcgatgacaaaccgcccgctttctgaagtcaatcagcattcacaactgatctccaggcttgtccaggtcatcgaagattcattccagatgcaagtcaacagggaaagcgtgaactatttgcggctgatcaggcacttgcgctttacgattgacaggataaaacgggacgagccgattcaggaaccggaaaaattaatgttgttgttgaaaacggaatatccgctgtgttacaatactgcttggaagatgatcaagatcttgcagcaagcgctcaagaaaccggttcatgaggcagaagccgtttatttgacattgcatttgtaccgtttgactaataaaatttcataa